European Patent Specification EP 3 532 628 B1, published February 28, 2024. Title: METHOD FOR PRODUCING OBJECTIVE SUBSTANCE. Applicant: Ajinomoto Co., Inc. The sequence listing filed with the application follows.

SEQUENCE LISTING (151 sequences)

SEQ ID NO: 1 - DNA, 1053 bp, Escherichia coli
atgaattatcagaacgacgatttacgcatcaaagaaatcaaagagttacttcctcctgtcgcattgctggaaaaattccccgctactgaaaatgccgcgaatacggttgcccatgcccgaaaagcgatccataagatcctgaaaggtaatgatgatcgcctgttggttgtgattggcccatgctcaattcatgatcctgtcgcggcaaaagagtatgccactcgcttgctggcgctgcgtgaagagctgaaagatgagctggaaatcgtaatgcgcgtctattttgaaaagccgcgtaccacggtgggctggaaagggctgattaacgatccgcatatggataatagcttccagatcaacgacggtctgcgtatagcccgtaaattgctgcttgatattaacgacagcggtctgccagcggcaggtgagtttctcgatatgatcaccccacaatatctcgctgacctgatgagctggggcgcaattggcgcacgtaccaccgaatcgcaggtgcaccgcgaactggcatcagggctttcttgtccggtcggcttcaaaaatggcaccgacggtacgattaaagtggctatcgatgccattaatgccgccggtgcgccgcactgcttcctgtccgtaacgaaatgggggcattcggcgattgtgaataccagcggtaacggcgattgccatatcattctgcgcggcggtaaagagcctaactacagcgcgaagcacgttgctgaagtgaaagaagggctgaacaaagcaggcctgccagcacaggtgatgatcgatttcagccatgctaactcgtccaaacaattcaaaaagcagatggatgtttgtgctgacgtttgccagcagattgccggtggcgaaaaggccattattggcgtgatggtggaaagccatctggtggaaggcaatcagagcctcgagagcggggagccgctggcctacggtaagagcatcaccgatgcctgcatcggctgggaagataccgatgctctgttacgtcaactggcgaatgcagtaaaagcgcgtcgcgggtaa

SEQ ID NO: 2 - protein, 350 aa, Escherichia coli
MNYQNDDLRIKEIKELLPPVALLEKFPATENAANTVAHARKAIHKILKGNDDRLLVVIGPCSIHDPVAAKEYATRLLALREELKDELEIVMRVYFEKPRTTVGWKGLINDPHMDNSFQINDGLRIARKLLLDINDSGLPAAGEFLDMITPQYLADLMSWGAIGARTTESQVHRELASGLSCPVGFKNGTDGTIKVAIDAINAAGAPHCFLSVTKWGHSAIVNTSGNGDCHIILRGGKEPNYSAKHVAEVKEGLNKAGLPAQVMIDFSHANSSKQFKKQMDVCADVCQQIAGGEKAIIGVMVESHLVEGNQSLESGEPLAYGKSITDACIGWEDTDALLRQLANAVKARRG

SEQ ID NO: 3 - DNA, 1089 bp, Escherichia coli
atggagaggattgtcgttactctcggggaacgtagttacccaattaccatcgcatctggtttgtttaatgaaccagcttcattcttaccgctgaaatcgggcgagcaggtcatgttggtcaccaacgaaaccctggctcctctgtatctcgataaggtccgcggcgtacttgaacaggcgggtgttaacgtcgatagcgttatcctccctgacggcgagcagtataaaagcctggctgtactcgataccgtctttacggcgttgttacaaaaaccgcatggtcgcgatactacgctggtggcgcttggcggcggcgtagtgggcgatctgaccggcttcgcggcggcgagttatcagcgcggtgtccgtttcattcaagtcccgacgacgttactgtcgcaggtcgattcctccgttggcggcaaaactgcggtcaaccatcccctcggtaaaaacatgattggcgcgttctaccaacctgcttcagtggtggtggatctcgactgtctgaaaacgcttcccccgcgtgagttagcgtcggggctggcagaagtcatcaaatacggcattattcttgacggtgcgttttttaactggctggaagagaatctggatgcgttgttgcgtctggacggtccggcaatggcgtactgtattcgccgttgttgtgaactgaaggcagaagttgtcgccgccgacgagcgcgaaaccgggttacgtgctttactgaatctgggacacacctttggtcatgccattgaagctgaaatggggtatggcaattggttacatggtgaagcggtcgctgcgggtatggtgatggcggcgcggacgtcggaacgtctcgggcagtttagttctgccgaaacgcagcgtattataaccctgctcaagcgggctgggttaccggtcaatgggccgcgcgaaatgtccgcgcaggcgtatttaccgcatatgctgcgtgacaagaaagtccttgcgggagagatgcgcttaattcttccgttggcaattggtaagagtgaagttcgcagcggcgtttcgcacgagcttgttcttaacgccattgccgattgtcaatcagcgtaa

SEQ ID NO: 4 - protein, 362 aa, Escherichia coli
MERIVVTLGERSYPITIASGLFNEPASFLPLKSGEQVMLVTNETLAPLYLDKVRGVLEQAGVNVDSVILPDGEQYKSLAVLDTVFTALLQKPHGRDTTLVALGGGVVGDLTGFAAASYQRGVRFIQVPTTLLSQVDSSVGGKTAVNHPLGKNMIGAFYQPASVVVDLDCLKTLPPRELASGLAEVIKYGIILDGAFFNWLEENLDALLRLDGPAMAYCIRRCCELKAEVVAADERETGLRALLNLGHTFGHAIEAEMGYGNWLHGEAVAAGMVMAARTSERLGQFSSAETQRIITLLKRAGLPVNGPREMSAQAYLPHMLRDKKVLAGEMRLILPLAIGKSEVRSGVSHELVLNAIADCQSA

SEQ ID NO: 5 - DNA, 759 bp, Escherichia coli
atgaaaaccgtaactgtaaaagatctcgtcattggtacgggcgcacctaaaatcatcgtctcgctgatggcgaaagatatcgccagcgtgaaatccgaagctctcgcctatcgtgaagcggactttgatattctggaatggcgtgtggaccactatgccgacctctccaatgtggagtctgtcatggcggcagcaaaaattctccgtgagaccatgccagaaaaaccgctgctgtttaccttccgcagtgccaaagaaggcggcgagcaggcgatttccaccgaggcttatattgcactcaatcgtgcagccatcgacagcggcctggttgatatgatcgatctggagttatttaccggtgatgatcaggttaaagaaaccgtcgcctacgcccacgcgcatgatgtgaaagtagtcatgtccaaccatgacttccataaaacgccggaagccgaagaaatcattgcccgtctgcgcaaaatgcaatccttcgacgccgatattcctaagattgcgctgatgccgcaaagtaccagcgatgtgctgacgttgcttgccgcgaccctggagatgcaggagcagtatgccgatcgtccaattatcacgatgtcgatggcaaaaactggcgtaatttctcgtctggctggtgaagtatttggctcggcggcaacttttggtgcggtaaaaaaagcgtctgcgccagggcaaatctcggtaaatgatttgcgcacggtattaactattttacaccaggcataa

SEQ ID NO: 6 - protein, 252 aa, Escherichia coli
MKTVTVKDLVIGTGAPKIIVSLMAKDIASVKSEALAYREADFDILEWRVDHYADLSNVESVMAAAKILRETMPEKPLLFTFRSAKEGGEQAISTEAYIALNRAAIDSGLVDMIDLELFTGDDQVKETVAYAHAHDVKVVMSNHDFHKTPEAEEIIARLRKMQSFDADIPKIALMPQSTSDVLTLLAATLEMQEQYADRPIITMSMAKTGVISRLAGEVFGSAATFGAVKKASAPGQISVNDLRTVLTILHQA

SEQ ID NO: 7 - DNA, 843 bp, Bacillus thuringiensis
atgaaatattcgctatgtaccatttcatttcgtcatcaattaatttcatttactgatattgttcaatttgcatatgaaaacggttttgaaggaattgaattatgggggacgcatgcacaaaatttgtacatgcaagaacgtgaaacgacagaacgagaattgaattttctaaaggataaaaacttagaaattacgatgataagtgattacttagatatatcattatcagcagattttgaaaaaacgatagagaaaagtgaacaacttgtagtactagctaattggtttaatacgaataaaattcgcacgtttgctgggcaaaaagggagcaaggacttctcggaacaagagagaaaagagtatgtgaagcgaatacgtaagatttgtgatgtgtttgctcagaacaatatgtatgtgctgttagaaacacatcccaatacactaacggacacattgccttctactatagagttattagaagaagtaaaccatccgaatttaaaaataaatcttgattttcttcatatatgggagtctggcgcagatccaatagacagtttccatcgattaaagccgtggacactacattaccattttaagaatatatcttcagcggattatttgcatgtgtttgaacctaataatgtatatgctgcagcaggaagtcgtataggtatggttccgttatttgaaggtattgtaaattatgatgagattattcaggaagtgagaaatacggatctttttgcttccttagaatggtttggacataattcaaaagagatattaaaagaagaaatgaaagtattaataaatagaaaattagaagtagtaacttcgtaa

SEQ ID NO: 8 - protein, 280 aa, Bacillus thuringiensis
MKYSLCTISFRHQLISFTDIVQFAYENGFEGIELWGTHAQNLYMQERETTERELNFLKDKNLEITMISDYLDISLSADFEKTIEKSEQLVVLANWFNTNKIRTFAGQKGSKDFSEQERKEYVKRIRKICDVFAQNNMYVLLETHPNTLTDTLPSTIELLEEVNHPNLKINLDFLHIWESGADPIDSFHRLKPWTLHYHFKNISSADYLHVFEPNNVYAAAGSRIGMVPLFEGIVNYDEIIQEVRNTDLFASLEWFGHNSKEILKEEMKVLINRKLEVVTS

SEQ ID NO: 9 - DNA, 1542 bp, Escherichia coli
atgcgtctggaagtcttttgtgaagaccgactcggtctgacccgcgaattactcgatctactcgtgctaagaggcattgatttacgcggtattgagattgatcccattgggcgaatctacctcaattttgctgaactggagtttgagagtttcagcagtctgatggccgaaatacgccgtattgcgggtgttaccgatgtgcgtactgtcccgtggatgccttccgaacgtgagcatctggcgttgagcgcgttactggaggcgttgcctgaacctgtgctctctgtcgatatgaaaagcaaagtggatatggcgaacccggcgagctgtcagctttttgggcaaaaattggatcgcctgcgcaaccataccgccgcacaattgattaacggctttaattttttacgttggctggaaagcgaaccgcaagattcgcataacgagcatgtcgttattaatgggcagaatttcctgatggagattacgcctgtttatcttcaggatgaaaatgatcaacacgtcctgaccggtgcggtggtgatgttgcgatcaacgattcgtatgggccgccagttgcaaaatgtcgccgcccaggacgtcagcgccttcagtcaaattgtcgccgtcagcccgaaaatgaagcatgttgtcgaacaggcgcagaaactggcgatgctaagcgcgccgctgctgattacgggtgacacaggtacaggtaaagatctctttgcctacgcctgccatcaggcaagccccagagcgggcaaaccttacctggcgctgaactgtgcgtctataccggaagatgcggtcgagagtgaactgtttggtcatgctccggaagggaagaaaggattctttgagcaggcgaacggtggttcggtgctgttggatgaaataggggaaatgtcaccacggatgcaggcgaaattactgcgtttccttaatgatggcactttccgtcgggttggcgaagaccatgaggtgcatgtcgatgtgcgggtgatttgcgctacgcagaagaatctggtcgaactggtgcaaaaaggcatgttccgtgaagatctctattatcgtctgaacgtgttgacgctcaatctgccgccgctacgtgactgtccgcaggacatcatgccgttaactgagctgttcgtcgcccgctttgccgacgagcagggcgtgccgcgtccgaaactggccgctgacctgaatactgtacttacgcgttatgcgtggccgggaaatgtgcggcagttaaagaacgctatctatcgcgcactgacacaactggacggttatgagctgcgtccacaggatattttgttgccggattatgacgccgcaacggtagccgtgggcgaagatgcgatggaaggttcgctggacgaaatcaccagccgttttgaacgctcggtattaacccagctttatcgcaattatcccagcacgcgcaaactggcaaaacgtctcggcgtttcacataccgcgattgccaataagttgcgggaatatggtctgagtcagaagaagaacgaagagtaa

SEQ ID NO: 10 - protein, 513 aa, Escherichia coli
MRLEVFCEDRLGLTRELLDLLVLRGIDLRGIEIDPIGRIYLNFAELEFESFSSLMAEIRRIAGVTDVRTVPWMPSEREHLALSALLEALPEPVLSVDMKSKVDMANPASCQLFGQKLDRLRNHTAAQLINGFNFLRWLESEPQDSHNEHVVINGQNFLMEITPVYLQDENDQHVLTGAVVMLRSTIRMGRQLQNVAAQDVSAFSQIVAVSPKMKHVVEQAQKLAMLSAPLLITGDTGTGKDLFAYACHQASPRAGKPYLALNCASIPEDAVESELFGHAPEGKKGFFEQANGGSVLLDEIGEMSPRMQAKLLRFLNDGTFRRVGEDHEVHVDVRVICATQKNLVELVQKGMFREDLYYRLNVLTLNLPPLRDCPQDIMPLTELFVARFADEQGVPRPKLAADLNTVLTRYAWPGNVRQLKNAIYRALTQLDGYELRPQDILLPDYDAATVAVGEDAMEGSLDEITSRFERSVLTQLYRNYPSTRKLAKRLGVSHTAIANKLREYGLSQKKNEE

SEQ ID NO: 11 - DNA, 2304 bp, Homo sapiens
cggcctgcgtccgccaccggaagcgccctcctaatccccgcagcgccaccgccattgccgccatcgtcgtggggcttctggggcagctagggctgcccgccgcgctgcctgcgccggaccggggcgggtccagtcccgggcgggccgtcgcgggagagaaataacatctgctttgctgccgagctcagaggagaccccagacccctcccgcagccagagggctggagcctgctcagaggtgctttgaagatgccggaggccccgcctctgctgttggcagctgtgttgctgggcctggtgctgctggtggtgctgctgctgcttctgaggcactggggctggggcctgtgccttatcggctggaacgagttcatcctgcagcccatccacaacctgctcatgggtgacaccaaggagcagcgcatcctgaaccacgtgctgcagcatgcggagcccgggaacgcacagagcgtgctggaggccattgacacctactgcgagcagaaggagtgggccatgaacgtgggcgacaagaaaggcaagatcgtggacgccgtgattcaggagcaccagccctccgtgctgctggagctgggggcctactgtggctactcagctgtgcgcatggcccgcctgctgtcaccaggggcgaggctcatcaccatcgagatcaaccccgactgtgccgccatcacccagcggatggtggatttcgctggcgtgaaggacaaggtcacccttgtggttggagcgtcccaggacatcatcccccagctgaagaagaagtatgatgtggacacactggacatggtcttcctcgaccactggaaggaccggtacctgccggacacgcttctcttggaggaatgtggcctgctgcggaaggggacagtgctactggctgacaacgtgatctgcccaggtgcgccagacttcctagcacacgtgcgcgggagcagctgctttgagtgcacacactaccaatcgttcctggaatacagggaggtggtggacggcctggagaaggccatctacaagggcccaggcagcgaagcagggccctgactgcccccccggcccccctctcgggctctctcacccagcctggtactgaaggtgccagacgtgctcctgctgaccttctgcggctccgggctgtgtcctaaatgcaaagcacacctcggccgaggcctgcgccctgacatgctaacctctctgaactgcaacactggattgttcttttttaagactcaatcatgacttctttactaacactggctagctatattatcttatatactaatatcatgttttaaaaatataaaatagaaattaagaatctaaatatttagatataactcgacttagtacatccttctcaactgccattcccctgctgcccttgacttgggcaccaaacattcaaagctccccttgacggacgctaacgctaagggcggggcccctagctggctgggttctgggtggcacgcctggcccactggcctcccagccacagtggtgcagaggtcagccctcctgcagctaggccaggggcacctgttagccccatggggacgactgccggcctgggaaacgaagaggagtcagccagcattcacacctttctgaccaagcaggcgctggggacaggtggaccccgcagcagcaccagcccctctgggccccatgtggcacagagtggaagcatctccttccctactccccactgggccttgcttacagaagaggcaatggctcagaccagctcccgcatccctgtagttgcctccctggcccatgagtgaggatgcagtgctggtttctgcccacctacacctagagctgtccccatctcctccaaggggtcagactgctagccacctcagaggctccaagggcccagttcccaggcccaggacaggaatcaaccctgtgctagctgagttcacctgcaccgagaccagcccctagccaagattctactcctgggctcaaggcctggctagcccccagccagcccactcctatggatagacagaccagtgagcccaagtggacaagtttggggccacccagggaccagaaacagagcctctgcaggacacagcagatgggcacctgggaccacctccacccagggccctgccccagacgcgcagaggcccgacacaagggagaagccagccacttgtgccagacctgagtggcagaaagcaaaaagttcctttgctgctttaatttttaaattttcttacaaaaatttaggtgtttaccaatagtcttattttggcttatttttaa

SEQ ID NO: 12 - DNA, 2262 bp, Homo sapiens
ctcccacgggaggagcaagaacacagaacagagggggcaagacagctccaccaggagtcaggagtgaatcccctctgggaacgaggcactaggaagaagaacttccagcccaggagaaataacatctgctttgctgccgagctcagaggagaccccagacccctcccgcagccagagggctggagcctgctcagaggtgctttgaagatgccggaggccccgcctctgctgttggcagctgtgttgctgggcctggtgctgctggtggtgctgctgctgcttctgaggcactggggctggggcctgtgccttatcggctggaacgagttcatcctgcagcccatccacaacctgctcatgggtgacaccaaggagcagcgcatcctgaaccacgtgctgcagcatgcggagcccgggaacgcacagagcgtgctggaggccattgacacctactgcgagcagaaggagtgggccatgaacgtgggcgacaagaaaggcaagatcgtggacgccgtgattcaggagcaccagccctccgtgctgctggagctgggggcctactgtggctactcagctgtgcgcatggcccgcctgctgtcaccaggggcgaggctcatcaccatcgagatcaaccccgactgtgccgccatcacccagcggatggtggatttcgctggcgtgaaggacaaggtcacccttgtggttggagcgtcccaggacatcatcccccagctgaagaagaagtatgatgtggacacactggacatggtcttcctcgaccactggaaggaccggtacctgccggacacgcttctcttggaggaatgtggcctgctgcggaaggggacagtgctactggctgacaacgtgatctgcccaggtgcgccagacttcctagcacacgtgcgcgggagcagctgctttgagtgcacacactaccaatcgttcctggaatacagggaggtggtggacggcctggagaaggccatctacaagggcccaggcagcgaagcagggccctgactgcccccccggcccccctctcgggctctctcacccagcctggtactgaaggtgccagacgtgctcctgctgaccttctgcggctccgggctgtgtcctaaatgcaaagcacacctcggccgaggcctgcgccctgacatgctaacctctctgaactgcaacactggattgttcttttttaagactcaatcatgacttctttactaacactggctagctatattatcttatatactaatatcatgttttaaaaatataaaatagaaattaagaatctaaatatttagatataactcgacttagtacatccttctcaactgccattcccctgctgcccttgacttgggcaccaaacattcaaagctccccttgacggacgctaacgctaagggcggggcccctagctggctgggttctgggtggcacgcctggcccactggcctcccagccacagtggtgcagaggtcagccctcctgcagctaggccaggggcacctgttagccccatggggacgactgccggcctgggaaacgaagaggagtcagccagcattcacacctttctgaccaagcaggcgctggggacaggtggaccccgcagcagcaccagcccctctgggccccatgtggcacagagtggaagcatctccttccctactccccactgggccttgcttacagaagaggcaatggctcagaccagctcccgcatccctgtagttgcctccctggcccatgagtgaggatgcagtgctggtttctgcccacctacacctagagctgtccccatctcctccaaggggtcagactgctagccacctcagaggctccaagggcccagttcccaggcccaggacaggaatcaaccctgtgctagctgagttcacctgcaccgagaccagcccctagccaagattctactcctgggctcaaggcctggctagcccccagccagcccactcctatggatagacagaccagtgagcccaagtggacaagtttggggccacccagggaccagaaacagagcctctgcaggacacagcagatgggcacctgggaccacctccacccagggccctgccccagacgcgcagaggcccgacacaagggagaagccagccacttgtgccagacctgagtggcagaaagcaaaaagttcctttgctgctttaatttttaaattttcttacaaaaatttaggtgtttaccaatagtcttattttggcttatttttaa

SEQ ID NO: 13 - DNA, 2279 bp, Homo sapiens
tggagataacacggatcgctgtgtacactgtgtgctccggttgttgcatccgagggttgatcggatggtggttcccatccagatccaagtcctggcccctgatcacagagaaacacagctggacattaaagtgaaataacatctgctttgctgccgagctcagaggagaccccagacccctcccgcagccagagggctggagcctgctcagaggtgctttgaagatgccggaggccccgcctctgctgttggcagctgtgttgctgggcctggtgctgctggtggtgctgctgctgcttctgaggcactggggctggggcctgtgccttatcggctggaacgagttcatcctgcagcccatccacaacctgctcatgggtgacaccaaggagcagcgcatcctgaaccacgtgctgcagcatgcggagcccgggaacgcacagagcgtgctggaggccattgacacctactgcgagcagaaggagtgggccatgaacgtgggcgacaagaaaggcaagatcgtggacgccgtgattcaggagcaccagccctccgtgctgctggagctgggggcctactgtggctactcagctgtgcgcatggcccgcctgctgtcaccaggggcgaggctcatcaccatcgagatcaaccccgactgtgccgccatcacccagcggatggtggatttcgctggcgtgaaggacaaggtcacccttgtggttggagcgtcccaggacatcatcccccagctgaagaagaagtatgatgtggacacactggacatggtcttcctcgaccactggaaggaccggtacctgccggacacgcttctcttggaggaatgtggcctgctgcggaaggggacagtgctactggctgacaacgtgatctgcccaggtgcgccagacttcctagcacacgtgcgcgggagcagctgctttgagtgcacacactaccaatcgttcctggaatacagggaggtggtggacggcctggagaaggccatctacaagggcccaggcagcgaagcagggccctgactgcccccccggcccccctctcgggctctctcacccagcctggtactgaaggtgccagacgtgctcctgctgaccttctgcggctccgggctgtgtcctaaatgcaaagcacacctcggccgaggcctgcgccctgacatgctaacctctctgaactgcaacactggattgttcttttttaagactcaatcatgacttctttactaacactggctagctatattatcttatatactaatatcatgttttaaaaatataaaatagaaattaagaatctaaatatttagatataactcgacttagtacatccttctcaactgccattcccctgctgcccttgacttgggcaccaaacattcaaagctccccttgacggacgctaacgctaagggcggggcccctagctggctgggttctgggtggcacgcctggcccactggcctcccagccacagtggtgcagaggtcagccctcctgcagctaggccaggggcacctgttagccccatggggacgactgccggcctgggaaacgaagaggagtcagccagcattcacacctttctgaccaagcaggcgctggggacaggtggaccccgcagcagcaccagcccctctgggccccatgtggcacagagtggaagcatctccttccctactccccactgggccttgcttacagaagaggcaatggctcagaccagctcccgcatccctgtagttgcctccctggcccatgagtgaggatgcagtgctggtttctgcccacctacacctagagctgtccccatctcctccaaggggtcagactgctagccacctcagaggctccaagggcccagttcccaggcccaggacaggaatcaaccctgtgctagctgagttcacctgcaccgagaccagcccctagccaagattctactcctgggctcaaggcctggctagcccccagccagcccactcctatggatagacagaccagtgagcccaagtggacaagtttggggccacccagggaccagaaacagagcctctgcaggacacagcagatgggcacctgggaccacctccacccagggccctgccccagacgcgcagaggcccgacacaagggagaagccagccacttgtgccagacctgagtggcagaaagcaaaaagttcctttgctgctttaatttttaaattttcttacaaaaatttaggtgtttaccaatagtcttattttggcttatttttaa

SEQ ID NO: 14 - DNA, 2035 bp, Homo sapiens
gctgttggcagctgtgttgctgggcctggtgctgctggtggtgctgctgctgcttctgaggcactggggctggggcctgtgccttatcggctggaacgagttcatcctgcagcccatccacaacctgctcatgggtgacaccaaggagcagcgcatcctgaaccacgtgctgcagcatgcggagcccgggaacgcacagagcgtgctggaggccattgacacctactgcgagcagaaggagtgggccatgaacgtgggcgacaagaaaggcaagatcgtggacgccgtgattcaggagcaccagccctccgtgctgctggagctgggggcctactgtggctactcagctgtgcgcatggcccgcctgctgtcaccaggggcgaggctcatcaccatcgagatcaaccccgactgtgccgccatcacccagcggatggtggatttcgctggcgtgaaggacaaggtcacccttgtggttggagcgtcccaggacatcatcccccagctgaagaagaagtatgatgtggacacactggacatggtcttcctcgaccactggaaggaccggtacctgccggacacgcttctcttggaggaatgtggcctgctgcggaaggggacagtgctactggctgacaacgtgatctgcccaggtgcgccagacttcctagcacacgtgcgcgggagcagctgctttgagtgcacacactaccaatcgttcctggaatacagggaggtggtggacggcctggagaaggccatctacaagggcccaggcagcgaagcagggccctgactgcccccccggcccccctctcgggctctctcacccagcctggtactgaaggtgccagacgtgctcctgctgaccttctgcggctccgggctgtgtcctaaatgcaaagcacacctcggccgaggcctgcgccctgacatgctaacctctctgaactgcaacactggattgttcttttttaagactcaatcatgacttctttactaacactggctagctatattatcttatatactaatatcatgttttaaaaatataaaatagaaattaagaatctaaatatttagatataactcgacttagtacatccttctcaactgccattcccctgctgcccttgacttgggcaccaaacattcaaagctccccttgacggacgctaacgctaagggcggggcccctagctggctgggttctgggtggcacgcctggcccactggcctcccagccacagtggtgcagaggtcagccctcctgcagctaggccaggggcacctgttagccccatggggacgactgccggcctgggaaacgaagaggagtcagccagcattcacacctttctgaccaagcaggcgctggggacaggtggaccccgcagcagcaccagcccctctgggccccatgtggcacagagtggaagcatctccttccctactccccactgggccttgcttacagaagaggcaatggctcagaccagctcccgcatccctgtagttgcctccctggcccatgagtgaggatgcagtgctggtttctgcccacctacacctagagctgtccccatctcctccaaggggtcagactgctagccacctcagaggctccaagggcccagttcccaggcccaggacaggaatcaaccctgtgctagctgagttcacctgcaccgagaccagcccctagccaagattctactcctgggctcaaggcctggctagcccccagccagcccactcctatggatagacagaccagtgagcccaagtggacaagtttggggccacccagggaccagaaacagagcctctgcaggacacagcagatgggcacctgggaccacctccacccagggccctgccccagacgcgcagaggcccgacacaagggagaagccagccacttgtgccagacctgagtggcagaaagcaaaaagttcctttgctgctttaatttttaaattttcttacaaaaatttaggtgtttaccaatagtcttattttggcttatttttaa

SEQ ID NO: 15 - protein, 271 aa, Homo sapiens
MPEAPPLLLAAVLLGLVLLVVLLLLLRHWGWGLCLIGWNEFILQPIHNLLMGDTKEQRILNHVLQHAEPGNAQSVLEAIDTYCEQKEWAMNVGDKKGKIVDAVIQEHQPSVLLELGAYCGYSAVRMARLLSPGARLITIEINPDCAAITQRMVDFAGVKDKVTLVVGASQDIIPQLKKKYDVDTLDMVFLDHWKDRYLPDTLLLEECGLLRKGTVLLADNVICPGAPDFLAHVRGSSCFECTHYQSFLEYREVVDGLEKAIYKGPGSEAGP

SEQ ID NO: 16 - protein, 221 aa, Homo sapiens
MGDTKEQRILNHVLQHAEPGNAQSVLEAIDTYCEQKEWAMNVGDKKGKIVDAVIQEHQPSVLLELGAYCGYSAVRMARLLSPGARLITIEINPDCAAITQRMVDFAGVKDKVTLVVGASQDIIPQLKKKYDVDTLDMVFLDHWKDRYLPDTLLLEECGLLRKGTVLLADNVICPGAPDFLAHVRGSSCFECTHYQSFLEYREVVDGLEKAIYKGPGSEAGP

SEQ ID NO: 17 - DNA, 3453 bp, Nocardia brasiliensis
ttgttcgccgaggacgagcaggtgaaagccgcggtgccggaccaggaggtggtcgaggcgatccgggcgcccggcctgcgcctggcacagatcatggccaccgtgatggagcgctatgcggaccgccccgcggtgggacagcgggcgagcgagccggtcaccgagagcggtcgcaccaccttccggctgctcccggaattcgagaccctgacctaccgcgagctgtgggcgcgcgtccgcgcggtggccgccgcgtggcacggagatgccgaaaggcctttgcgggccggggatttcgttgctctgctgggtttcgccggcatcgattacggcaccctcgatctcgcgaacatccatctcggcctcgtcacggtgccgctgcaatccggcgccacggccccgcaactcgccgcgatcctggccgagaccacgccccgggtgctggccgcgacacccgaccatctcgatatcgccgtcgaattgctgaccgggggagcctcgccggaacggctggtggtattcgactaccgccccgcggacgacgatcaccgggcggcgctcgagtccgcgcgcagacggttgagcgacgcgggcagtgcggtggtggtcgagacgctcgacgcggtccgcgcccgcggcagcgaattgccggccgcgccgctgttcgttcccgccgcggacgaggacccgctggctctgctcatctacacctccggcagcaccggcacgcctaagggcgccatgtacaccgaaagactgaaccgcacgacgtggctgagcggggcgaaaggcgtcggcctcacgctcggctacatgccgatgagtcatattgccgggcgggcctcgttcgccggtgtgctggcccgcggcggcacggtctacttcaccgcccgcagcgatatgtcgacgctgttcgaagatctggccctggtgcggccgaccgagatgttcttcgtcccgcgcgtgtgcgacatgatcttccagcgctatcaggccgaactgtcgcggcgcgcgcccgccgcggccgcgagcccggaactcgagcaggaactgaagaccgaactgcgcttgtccgcggtcggggaccgcttactcggggcgatcgcgggcagcgcgccgctgtcggccgagatgcgggagttcatggagtcgctgctggatctggaactgcacgacggctacggctcgaccgaggcgggtatcggcgtactgcaagacaatatcgtccagcgtccgccggtcatcgattacaagctcgtcgacgtgccggaattgggctacttccggacggaccagccgcatccccgcggtgagttgctgttgaaaaccgaagggatgattccgggctacttccggcggcccgaggtgaccgcggagatcttcgacgaggacggtttctacaggaccggtgacatcgtcgccgaactcgaaccggatcggctgatctacctggaccgccgcaacaatgtgctgaaactggcccagggcgagttcgtcacggtcgcccatctggaagcggtgttcgcgaccagtccgctgatccggcagatctacatctacggcaacagcgagcgctcgttcctgctggcggtgatcgtgcccaccgcggacgcgctggccgacggtgtcaccgacgcgctgaacacggcgctgaccgaatccttgcgacagctcgcgaaagaagccgggctgcaatcctatgagctgccgcgcgagttcctggtcgaaaccgaaccgttcaccgtcgagaacggtctgctctccggtatcgcgaaactgttgcggcccaagctcaaggagcactacggcgagcgactcgagcagctgtaccgcgatatcgaggcgaaccgcaacgacgagctgatcgagctgcggcgcaccgcggccgagctgccggtgctcgaaaccgtcacgcgggctgcacgttcgatgctcggactggccgcgtcggagttgcggccggacgcgcatttcaccgatctcggcggtgattcactgtccgcgctgtcgttttcgaccctgctgcaggacatgctcgaggtcgaggtcccggtcggtgtcatcgtgagccccgccaactcgctcgccgatctggcgaaatacatcgaggccgaacggcattcgggggtgcggcggccgagcctgatctcggtgcacggtcccggcaccgagatccgtgccgccgatctcaccctggacaagttcatcgacgagcgcaccctcgctgccgcgaaagcggttccggccgcgccggcccaggcgcagaccgtcctgctcaccggggcgaacggctatctcggccgcttcctgtgcctggaatggctgcagcgactggaccagaccggcggcacgctggtctgcatcgtgcgcggtaccgacgcggccgccgcgcggaagcgcctggatgcggtgttcgacagcggtgatccggagctgctcgaccactaccggaagctggccgccgagcacctcgaggtgctcgcgggcgatatcggcgacccgaatctcggcctggacgaagcgacttggcagcggctcgccgcgaccgtcgacctgatcgtgcaccccgccgccctcgtcaaccatgtgctgccgtacagccagctgttcgggccgaatgtggtcggcaccgccgagatcatccggctggccatcaccgagcgccgtaagcccgtgacgtacctgtcgacggtcgcggtggccgcacaggtcgatcccgccggcttcgacgaggagcgcgatatccgggagatgagcgcggtgcgctccatcgacgccgggtacgcgaacggttacggcaacagcaagtgggccggcgaggtgctgctgcgcgaggcccatgatctgtgcgggctgccggtcgccgtgttccgctcggacatgatcctggcgcacagcaaatacgtcggtcagctcaacgtccccgatgtgttcacccggctcatcctgagcctggcgctcaccggcatcgcaccgtattcgttctacgggacggacagcgccgggcagcgcaggcgggcccactacgacggtctgcccgccgatttcgtcgccgaggcgatcaccaccctcggcgcgcgagccgagtcggggttccatacctacgacgtgtggaacccgtacgacgacggcatctcgctggacgaattcgtcgactggctcggcgatttcggcgtgccgatccagcggatcgacgactacgacgaatggttccggcgtttcgagaccgcgatccgcgcgctgcccgaaaagcagcgcgatgcttcgctgctaccgctgctggacgcacaccggcggccactgcgcgcggtgcgcggttcgctgttgcccgccaagaacttccaggcggcggtgcagtccgcgcggatcggccccgatcaggacatcccgcatctttccccgcagttgatcgacaagtacgtcaccgacctgcgccacctcggcctgctctga

SEQ ID NO: 18 - protein, 1150 aa, Nocardia brasiliensis
MFAEDEQVKAAVPDQEVVEAIRAPGLRLAQIMATVMERYADRPAVGQRASEPVTESGRTTFRLLPEFETLTYRELWARVRAVAAAWHGDAERPLRAGDFVALLGFAGIDYGTLDLANIHLGLVTVPLQSGATAPQLAAILAETTPRVLAATPDHLDIAVELLTGGASPERLVVFDYRPADDDHRAALESARRRLSDAGSAVVVETLDAVRARGSELPAAPLFVPAADEDPLALLIYTSGSTGTPKGAMYTERLNRTTWLSGAKGVGLTLGYMPMSHIAGRASFAGVLARGGTVYFTARSDMSTLFEDLALVRPTEMFFVPRVCDMIFQRYQAELSRRAPAAAASPELEQELKTELRLSAVGDRLLGAIAGSAPLSAEMREFMESLLDLELHDGYGSTEAGIGVLQDNIVQRPPVIDYKLVDVPELGYFRTDQPHPRGELLLKTEGMIPGYFRRPEVTAEIFDEDGFYRTGDIVAELEPDRLIYLDRRNNVLKLAQGEFVTVAHLEAVFATSPLIRQIYIYGNSERSFLLAVIVPTADALADGVTDALNTALTESLRQLAKEAGLQSYELPREFLVETEPFTVENGLLSGIAKLLRPKLKEHYGERLEQLYRDIEANRNDELIELRRTAAELPVLETVTRAARSMLGLAASELRPDAHFTDLGGDSLSALSFSTLLQDMLEVEVPVGVIVSPANSLADLAKYIEAERHSGVRRPSLISVHGPGTEIRAADLTLDKFIDERTLAAAKAVPAAPAQAQTVLLTGANGYLGRFLCLEWLQRLDQTGGTLVCIVRGTDAAAARKRLDAVFDSGDPELLDHYRKLAAEHLEVLAGDIGDPNLGLDEATWQRLAATVDLIVHPAALVNHVLPYSQLFGPNVVGTAEIIRLAITERRKPVTYLSTVAVAAQVDPAGFDEERDIREMSAVRSIDAGYANGYGNSKWAGEVLLREAHDLCGLPVAVFRSDMILAHSKYVGQLNVPDVFTRLILSLALTGIAPYSFYGTDSAGQRRRAHYDGLPADFVAEAITTLGARAESGFHTYDVWNPYDDGISLDEFVDWLGDFGVPIQRIDDYDEWFRRFETAIRALPEKQRDASLLPLLDAHRRPLRAVRGSLLPAKNFQAAVQSARIGPDQDIPHLSPQLIDKYVTDLRHLGLL

SEQ ID NO: 19 - DNA, 3501 bp, Nocardia brasiliensis
atggcgactgattcgcgaagcgatcggctacggcgtcgaattgcacagttgttcgccgaggacgagcaggtgaaagccgcggtgccggaccaggaggtggtcgaggcgatccgggcgcccggcctgcgcctggcacagatcatggccaccgtgatggagcgctatgcggaccgccccgcggtgggacagcgggcgagcgagccggtcaccgagagcggtcgcaccaccttccggctgctcccggaattcgagaccctgacctaccgcgagctgtgggcgcgcgtccgcgcggtggccgccgcgtggcacggagatgccgaaaggcctttgcgggccggggatttcgttgctctgctgggtttcgccggcatcgattacggcaccctcgatctcgcgaacatccatctcggcctcgtcacggtgccgctgcaatccggcgccacggccccgcaactcgccgcgatcctggccgagaccacgccccgggtgctggccgcgacacccgaccatctcgatatcgccgtcgaattgctgaccgggggagcctcgccggaacggctggtggtattcgactaccgccccgcggacgacgatcaccgggcggcgctcgagtccgcgcgcagacggttgagcgacgcgggcagtgcggtggtggtcgagacgctcgacgcggtccgcgcccgcggcagcgaattgccggccgcgccgctgttcgttcccgccgcggacgaggacccgctggctctgctcatctacacctccggcagcaccggcacgcctaagggcgccatgtacaccgaaagactgaaccgcacgacgtggctgagcggggcgaaaggcgtcggcctcacgctcggctacatgccgatgagtcatattgccgggcgggcctcgttcgccggtgtgctggcccgcggcggcacggtctacttcaccgcccgcagcgatatgtcgacgctgttcgaagatctggccctggtgcggccgaccgagatgttcttcgtcccgcgcgtgtgcgacatgatcttccagcgctatcaggccgaactgtcgcggcgcgcgcccgccgcggccgcgagcccggaactcgagcaggaactgaagaccgaactgcgcttgtccgcggtcggggaccgcttactcggggcgatcgcgggcagcgcgccgctgtcggccgagatgcgggagttcatggagtcgctgctggatctggaactgcacgacggctacggctcgaccgaggcgggtatcggcgtactgcaagacaatatcgtccagcgtccgccggtcatcgattacaagctcgtcgacgtgccggaattgggctacttccggacggaccagccgcatccccgcggtgagttgctgttgaaaaccgaagggatgattccgggctacttccggcggcccgaggtgaccgcggagatcttcgacgaggacggtttctacaggaccggtgacatcgtcgccgaactcgaaccggatcggctgatctacctggaccgccgcaacaatgtgctgaaactggcccagggcgagttcgtcacggtcgcccatctggaagcggtgttcgcgaccagtccgctgatccggcagatctacatctacggcaacagcgagcgctcgttcctgctggcggtgatcgtgcccaccgcggacgcgctggccgacggtgtcaccgacgcgctgaacacggcgctgaccgaatccttgcgacagctcgcgaaagaagccgggctgcaatcctatgagctgccgcgcgagttcctggtcgaaaccgaaccgttcaccgtcgagaacggtctgctctccggtatcgcgaaactgttgcggcccaagctcaaggagcactacggcgagcgactcgagcagctgtaccgcgatatcgaggcgaaccgcaacgacgagctgatcgagctgcggcgcaccgcggccgagctgccggtgctcgaaaccgtcacgcgggctgcacgttcgatgctcggactggccgcgtcggagttgcggccggacgcgcatttcaccgatctcggcggtgattcactgtccgcgctgtcgttttcgaccctgctgcaggacatgctcgaggtcgaggtcccggtcggtgtcatcgtgagccccgccaactcgctcgccgatctggcgaaatacatcgaggccgaacggcattcgggggtgcggcggccgagcctgatctcggtgcacggtcccggcaccgagatccgtgccgccgatctcaccctggacaagttcatcgacgagcgcaccctcgctgccgcgaaagcggttccggccgcgccggcccaggcgcagaccgtcctgctcaccggggcgaacggctatctcggccgcttcctgtgcctggaatggctgcagcgactggaccagaccggcggcacgctggtctgcatcgtgcgcggtaccgacgcggccgccgcgcggaagcgcctggatgcggtgttcgacagcggtgatccggagctgctcgaccactaccggaagctggccgccgagcacctcgaggtgctcgcgggcgatatcggcgacccgaatctcggcctggacgaagcgacttggcagcggctcgccgcgaccgtcgacctgatcgtgcaccccgccgccctcgtcaaccatgtgctgccgtacagccagctgttcgggccgaatgtggtcggcaccgccgagatcatccggctggccatcaccgagcgccgtaagcccgtgacgtacctgtcgacggtcgcggtggccgcacaggtcgatcccgccggcttcgacgaggagcgcgatatccgggagatgagcgcggtgcgctccatcgacgccgggtacgcgaacggttacggcaacagcaagtgggccggcgaggtgctgctgcgcgaggcccatgatctgtgcgggctgccggtcgccgtgttccgctcggacatgatcctggcgcacagcaaatacgtcggtcagctcaacgtccccgatgtgttcacccggctcatcctgagcctggcgctcaccggcatcgcaccgtattcgttctacgggacggacagcgccgggcagcgcaggcgggcccactacgacggtctgcccgccgatttcgtcgccgaggcgatcaccaccctcggcgcgcgagccgagtcggggttccatacctacgacgtgtggaacccgtacgacgacggcatctcgctggacgaattcgtcgactggctcggcgatttcggcgtgccgatccagcggatcgacgactacgacgaatggttccggcgtttcgagaccgcgatccgcgcgctgcccgaaaagcagcgcgatgcttcgctgctaccgctgctggacgcacaccggcggccactgcgcgcggtgcgcggttcgctgttgcccgccaagaacttccaggcggcggtgcagtccgcgcggatcggccccgatcaggacatcccgcatctttccccgcagttgatcgacaagtacgtcaccgacctgcgccacctcggcctgctctga

SEQ ID NO: 20 - protein, 1166 aa, Nocardia brasiliensis
MATDSRSDRLRRRIAQLFAEDEQVKAAVPDQEVVEAIRAPGLRLAQIMATVMERYADRPAVGQRASEPVTESGRTTFRLLPEFETLTYRELWARVRAVAAAWHGDAERPLRAGDFVALLGFAGIDYGTLDLANIHLGLVTVPLQSGATAPQLAAILAETTPRVLAATPDHLDIAVELLTGGASPERLVVFDYRPADDDHRAALESARRRLSDAGSAVVVETLDAVRARGSELPAAPLFVPAADEDPLALLIYTSGSTGTPKGAMYTERLNRTTWLSGAKGVGLTLGYMPMSHIAGRASFAGVLARGGTVYFTARSDMSTLFEDLALVRPTEMFFVPRVCDMIFQRYQAELSRRAPAAAASPELEQELKTELRLSAVGDRLLGAIAGSAPLSAEMREFMESLLDLELHDGYGSTEAGIGVLQDNIVQRPPVIDYKLVDVPELGYFRTDQPHPRGELLLKTEGMIPGYFRRPEVTAEIFDEDGFYRTGDIVAELEPDRLIYLDRRNNVLKLAQGEFVTVAHLEAVFATSPLIRQIYIYGNSERSFLLAVIVPTADALADGVTDALNTALTESLRQLAKEAGLQSYELPREFLVETEPFTVENGLLSGIAKLLRPKLKEHYGERLEQLYRDIEANRNDELIELRRTAAELPVLETVTRAARSMLGLAASELRPDAHFTDLGGDSLSALSFSTLLQDMLEVEVPVGVIVSPANSLADLAKYIEAERHSGVRRPSLISVHGPGTEIRAADLTLDKFIDERTLAAAKAVPAAPAQAQTVLLTGANGYLGRFLCLEWLQRLDQTGGTLVCIVRGTDAAAARKRLDAVFDSGDPELLDHYRKLAAEHLEVLAGDIGDPNLGLDEATWQRLAATVDLIVHPAALVNHVLPYSQLFGPNVVGTAEIIRLAITERRKPVTYLSTVAVAAQVDPAGFDEERDIREMSAVRSIDAGYANGYGNSKWAGEVLLREAHDLCGLPVAVFRSDMILAHSKYVGQLNVPDVFTRLILSLALTGIAPYSFYGTDSAGQRRRAHYDGLPADFVAEAITTLGARAESGFHTYDVWNPYDDGISLDEFVDWLGDFGVPIQRIDDYDEWFRRFETAIRALPEKQRDASLLPLLDAHRRPLRAVRGSLLPAKNFQAAVQSARIGPDQDIPHLSPQLIDKYVTDLRHLGLL

SEQ ID NO: 21 - DNA, 621 bp, Escherichia coli
atgaaaactacgcatacctccctcccctttgccggacatacgctgcattttgttgagttcgatccggcgaatttttgtgagcaggatttactctggctgccgcactacgcacaactgcaacacgctggacgtaaacgtaaaacagagcatttagccggacggatcgctgctgtttatgctttgcgggaatatggctataaatgtgtgcccgcaatcggcgagctacgccaacctgtctggcctgcggaggtatacggcagtattagccactgtgggactacggcattagccgtggtatctcgtcaaccgattggcattgatatagaagaaattttttctgtacaaaccgcaagagaattgacagacaacattattacaccagcggaacacgagcgactcgcagactgcggtttagccttttctctggcgctgacactggcattttccgccaaagagagcgcatttaaggcaagtgagatccaaactgatgcaggttttctggactatcagataattagctggaataaacagcaggtcatcattcatcgtgagaatgagatgtttgctgtgcactggcagataaaagaaaagatagtcataacgctgtgccaacacgattaa

SEQ ID NO: 22 - protein, 206 aa, Escherichia coli
MKTTHTSLPFAGHTLHFVEFDPANFCEQDLLWLPHYAQLQHAGRKRKTEHLAGRIAAVYALREYGYKCVPAIGELRQPVWPAEVYGSISHCGTTALAVVSRQPIGIDIEEIFSVQTARELTDNIITPAEHERLADCGLAFSLALTLAFSAKESAFKASEIQTDAGFLDYQIISWNKQQVIIHRENEMFAVHWQIKEKIVITLCQHD

SEQ ID NO: 23 - DNA, 654 bp, Corynebacterium glutamicum
atgctggatgagtctttgtttccaaattcggcaaagttttctttcattaaaactggcgatgctgttaatttagaccatttccatcagttgcatccgttggaaaaggcactggtagcgcactcggttgatattagaaaagcagagtttggagatgccaggtggtgtgcacatcaggcactccaagctttgggacgagatagcggtgatcccattttgcgtggggaacgaggaatgccattgtggccttcttcggtgtctggttcattgacccacactgacggattccgagctgctgttgtggcgccacgattgttggtgcgttctatgggattggatgccgaacctgcggagccgttgcccaaggatgttttgggttcaatcgctcgggtgggggagattcctcaacttaagcgcttggaggaacaaggtgtgcactgcgcggatcgcctgctgttttgtgccaaggaagcaacatacaaagcgtggttcccgctgacgcataggtggcttggttttgaacaagctgagatcgacttgcgtgatgatggcacttttgtgtcctatttgctggttcgaccaactccagtgccgtttatttcaggtaaatgggtactgcgtgatggttatgtcatagctgcgactgcagtgacttga

SEQ ID NO: 24 - protein, 217 aa, Corynebacterium glutamicum
MLDESLFPNSAKFSFIKTGDAVNLDHFHQLHPLEKALVAHSVDIRKAEFGDARWCAHQALQALGRDSGDPILRGERGMPLWPSSVSGSLTHTDGFRAAVVAPRLLVRSMGLDAEPAEPLPKDVLGSIARVGEIPQLKRLEEQGVHCADRLLFCAKEATYKAWFPLTHRWLGFEQAEIDLRDDGTFVSYLLVRPTPVPFISGKWVLRDGYVIAATAVT

SEQ ID NO: 25 - DNA, 1428 bp, Corynebacterium glutamicum
atgcgcctgcgtgtctcgagtagtctcctccccttcctcgtccccaacctcgaccattacggtcgccctctcctaaaggagcctggcatggatatccgccaaacaattaacgacacagcaatgtcgagatatcagtggttcattgtatttatcgcagtgctgctcaacgcactggacggctttgatgtcctcgccatgtcttttactgcgaatgcagtgaccgaagaatttggactgagtggcagccagcttggtgtgctgctgagttccgcgctgttcggcatgaccgctggatctttgctgttcggtccgatcggtgaccgtttcggccgtaagaatgccctgatgatcgcgctgctgttcaacgtggtgggattggtattgtccgccaccgcgcagtccgcaggccagttgggcgtgtggcgtttgatcactggtatcggcatcggcggaatcctcgcctgcatcacagtggtgatcagtgagttctccaacaacaaaaaccgcggcatggccatgtccatctacgctgctggttacggcatcggcgcgtccttgggcggattcggcgcagcgcagctcatcccaacatttggatggcgctccgtgttcgcagccggtgcgatcgcaactggtatcgccaccatcgctactttcttcttcctgccagaatccgttgattggctgagcactcgccgccctgcgggcgctcgcgacaagatcaattacattgcgcgccgcctgggcaaagtcggtacctttgagcttccaggcgaacaaagcttgtcgacgaaaaaagccggtctccaatcgtatgcagtgctcgttaacaaagagaaccgtggaaccagcatcaagctgtgggttgcgttcggcatcgtgatgttcggcttctacttcgccaacacttggaccccgaagctgctcgtggaaaccggaatgtcagaacagcagggcatcatcggtggtttgatgttgtccatgggtggagcattcggttccctgctctacggtttcctcaccaccaagttcagctcccgaaacacactgatgaccttcatggtgctgtccggcctgacgctgatcctgttcatttcctccacctctgttccatccatcgcgtttgccagcggcgttgtcgtgggcatgctgatcaatggttgtgtggctggtctgtacaccctgtccccacagctgtactccgctgaagtacgcaccactggtgtgggcgctgcgattggtatgggtcgtgtcggtgcgatttccgcgccactgctggtgggtagcctgctggattctggctggtccccaacgcagctgtatgttggtgtggcagtgattgttattgccggtgcaaccgcattgattgggatgcgcactcaggcagtagccgtcgaaaagcagcctgaagccctagcgaccaaatag

SEQ ID NO: 26 - protein, 475 aa, Corynebacterium glutamicum
MRLRVSSSLLPFLVPNLDHYGRPLLKEPGMDIRQTINDTAMSRYQWFIVFIAVLLNALDGFDVLAMSFTANAVTEEFGLSGSQLGVLLSSALFGMTAGSLLFGPIGDRFGRKNALMIALLFNVVGLVLSATAQSAGQLGVWRLITGIGIGGILACITVVISEFSNNKNRGMAMSIYAAGYGIGASLGGFGAAQLIPTFGWRSVFAAGAIATGIATIATFFFLPESVDWLSTRRPAGARDKINYIARRLGKVGTFELPGEQSLSTKKAGLQSYAVLVNKENRGTSIKLWVAFGIVMFGFYFANTWTPKLLVETGMSEQQGIIGGLMLSMGGAFGSLLYGFLTTKFSSRNTLMTFMVLSGLTLILFISSTSVPSIAFASGVVVGMLINGCVAGLYTLSPQLYSAEVRTTGVGAAIGMGRVGAISAPLLVGSLLDSGWSPTQLYVGVAVIVIAGATALIGMRTQAVAVEKQPEALATK

SEQ ID NO: 27 - DNA, 1296 bp, Corynebacterium glutamicum
gtgtcaacgaccaccccaacccgcgcaaccaaaagtgtcggaacagttctcgcactcctgtggttcgcaattgtcctcgacggctttgacctagtcgtcctgggcgcaacaatcccgtccatgctggaggatcccgcgtgggatctcactgctggacaggccacacagatttccaccatcggcctcgtcggcatgaccatcggcgcactgaccattggtttcttaactgaccgtctgggtcgacgccgcgtcatgctgttctctgtggcagtgttttctgtattcaccctcctgctggcattcaccaccaacgtccagctcttcagcctgtggcgtttcctcgcaggtgttggccttggtggagcactccccaccgcaattgccatggtgaccgagtttcgccccggcaccaaagcgggctctgcatcaactaccttgatgaccggataccacgtcggggcagtagcaaccgctttccttggtctcttccttatcgacggctttggttggcactccatgttcatcgcaggcgctgtgccaggactactcctgctgccactgctgtatttcttccttccagaatccccgcagtacctcaaaatctccggcaagttggatgaggcgcaggcagttgcagcatcttatggactttccctggatgatgatcttgatcgcgaacacgaagaagaacttggcgagtcctcctcactttcctccctgttcaagccctcgttccgccgcaacaccctggcgatttggggcacctcattcatgggactcctcctggtctacggcctgaacacatggctgccacaaatcatgcgccaagcagactacgacatgggtaactccctgggcttcctcatggttcttaacatcggcgcagtgatcggcctttatattgcagggcgaattgccgataagaactcccctcgcaaaacagcactcgtatggttcgtgttctctgcatttttcctcgcactacttgctgtccggatgccactgatcggtctgtatggcatcgtgctgctcaccggcatctttgtgttcagctcccaggtactcatctacgccttcgttggtgagaatcaccctgccaagatgcgtgcaactgccatgggattctccgcaggaattggtcgcctcggcgcgatctcgggtccgttgctgggcggcctgcttgtcagtgccaaccttgcttacccatggggcttcttcgccttcgctggcgttggactgctgggcgcgctgattttctccgcatcgaagactctgaggcatcgcgagaacgcttag

SEQ ID NO: 28 - protein, 431 aa, Corynebacterium glutamicum
MSTTTPTRATKSVGTVLALLWFAIVLDGFDLVVLGATIPSMLEDPAWDLTAGQATQISTIGLVGMTIGALTIGFLTDRLGRRRVMLFSVAVFSVFTLLLAFTTNVQLFSLWRFLAGVGLGGALPTAIAMVTEFRPGTKAGSASTTLMTGYHVGAVATAFLGLFLIDGFGWHSMFIAGAVPGLLLLPLLYFFLPESPQYLKISGKLDEAQAVAASYGLSLDDDLDREHEEELGESSSLSSLFKPSFRRNTLAIWGTSFMGLLLVYGLNTWLPQIMRQADYDMGNSLGFLMVLNIGAVIGLYIAGRIADKNSPRKTALVWFVFSAFFLALLAVRMPLIGLYGIVLLTGIFVFSSQVLIYAFVGENHPAKMRATAMGFSAGIGRLGAISGPLLGGLLVSANLAYPWGFFAFAGVGLLGALIFSASKTLRHRENA

SEQ ID NO: 29 - DNA, 1131 bp, Corynebacterium glutamicum
atgacactgtccgaacgcaagctcaccaccaccgccaagattcttccccacccactcaacgcctggtacgtcgccgcttgggattatgaagtcacatctaaaaagcccatggccaggacaatcgccaacaaaccactcgctttgtaccgcaccaaagatggccgagccgttgcccttgcagacgcctgctggcaccgcctcgcaccgctatccaagggaaaactcgtgggcacagacggaatccaatgcccttatcacggcttggagtacaactccgcgggccgctgcatgaaaatgcccgcgcaggaaaccctcaacccgtcagcagccgtcaactcctaccccgtggtggaagcccaccgctttgtgtgggtgtggctgggcgatcccacattggcagatcccacccaagtacccgatatgcaccagatgagccaccccgaatgggcaggcgatggacgcaccatctccgctgactgcaactaccaattagtgctggacaacttgatggacctcacccacgaagaattcgtgcactcctccagcatcggccaagacgaacttagtgaatcagagttcgtggtcacccacactgaagattccgtgacggtcacccgctggatgcatgacatagatgcaccaccgttttggcaaaagaacatgaatgataagttcccaggatttgaaggcaaggtggatcgttggcagatcatccactactactacccttccaccatctgcattgatgttggtgtagcaaaggctggaaccggcgcgcaggaaggcgaccgcagccagggcgttaatgggtatgtaatgaacaccattaccccagattcagatcgttcctctcattacttctgggcattcatgcgcaactaccgcctggaaagccaaaccatcaccacccagctgcgcgacggtgtatccggtgtattcaaagaagacgaagacatgctgaccgctcagcaagatgccatcgacgccaacaccgactatgagttttacagcctcaacattgatgccggtggcatgtgggtgcgccgaatcctcgaggaagcactctccaaggaaggccgactggatatccccaccacattcccccgcgcaacaccgaagccggaggcataa

SEQ ID NO: 30 - protein, 376 aa, Corynebacterium glutamicum
MTLSERKLTTTAKILPHPLNAWYVAAWDYEVTSKKPMARTIANKPLALYRTKDGRAVALADACWHRLAPLSKGKLVGTDGIQCPYHGLEYNSAGRCMKMPAQETLNPSAAVNSYPVVEAHRFVWVWLGDPTLADPTQVPDMHQMSHPEWAGDGRTISADCNYQLVLDNLMDLTHEEFVHSSSIGQDELSESEFVVTHTEDSVTVTRWMHDIDAPPFWQKNMNDKFPGFEGKVDRWQIIHYYYPSTICIDVGVAKAGTGAQEGDRSQGVNGYVMNTITPDSDRSSHYFWAFMRNYRLESQTITTQLRDGVSGVFKEDEDMLTAQQDAIDANTDYEFYSLNIDAGGMWVRRILEEALSKEGRLDIPTTFPRATPKPEA

SEQ ID NO: 31 - DNA, 978 bp, Corynebacterium glutamicum
atgaactcgcaatggcaagatgcacatgttgtttccagcgaaatcatcgctgcagacattcgacgaatagaactatccccgaaatttgcgattccagtaaaacccggcgaacatctcaagatcatggtgcccctaaaaactggacaggaaaagagatcgtactccatcgttgacgctcgtcacgacggttcgactctcgccctgagcgtactcaaaaccagaaactcccgtggaggatctgagttcatgcatacgcttcgagctggagacacagttactgtctccaggccgtctcaggattttcctctccgcgtgggtgcgcctgagtatgtacttgttgccggcggaattggaatcacagcgatccgttcaatggcatctttattaaagaaattgggagcaaactaccgcattcatttcgcagcacgcagccttgatgccatggcttacaaagatgagctcgtggcagaacacggcgacaagctgcacctgcatctagattctgaaggcaccaccatcgatgtcccagcattgatcgaaaccttaaacccccacactgagctttatatgtgcggccccatccgcttgatggatgccatccggcgcgcatggaacacccgcggacttgaccccaccaatctgcgtttcgaaacgtttggaaacagtggatggttctccccagaggttttccacatccaagtaccagagctggggcttcacgccacagtcaacaaggatgaaagcatgctggaggctttgcaaaaggctggggcgaatatgatgtttgattgtcgaaaaggcgaatgtggtttgtgccaggttcgcgttctagaagtcgatggccaggttgatcaccgcgatgtgttcttctctgatcgtcaaaaagaatccgacgcaaaggcatgcgcctgcgtgtctcgagtagtctcctccccttcctcgtccccaacctcgaccattacggtcgccctctcctaa

SEQ ID NO: 32 - protein, 325 aa, Corynebacterium glutamicum
MNSQWQDAHVVSSEIIAADIRRIELSPKFAIPVKPGEHLKIMVPLKTGQEKRSYSIVDARHDGSTLALSVLKTRNSRGGSEFMHTLRAGDTVTVSRPSQDFPLRVGAPEYVLVAGGIGITAIRSMASLLKKLGANYRIHFAARSLDAMAYKDELVAEHGDKLHLHLDSEGTTIDVPALIETLNPHTELYMCGPIRLMDAIRRAWNTRGLDPTNLRFETFGNSGWFSPEVFHIQVPELGLHATVNKDESMLEALQKAGANMMFDCRKGECGLCQVRVLEVDGQVDHRDVFFSDRQKESDAKACACVSRVVSSPSSSPTSTITVALS

SEQ ID NO: 33 - DNA, 615 bp, Corynebacterium glutamicum
atgattgatacagggaagaacggcgagttccgctacgagcagtcgaatatcatcgatcagaacgaagccgagttcggcatcactccttcacagaccgtgggcccttacgtccacatcggtttgacccttgaaggtgcggagcatctcgtggagccaggttcggaaggcgcggtgtcctttactgtttccgcaactgatggcaacggcgaccccatcgcggatgccatgtttgaactgtggcaggccgatccagagggcatccacaactctgatttggatccaaaccgcacagcaccagcaaccgcagatggcttccgcgggcttggtcgcgcgatggcaaacgcgcagggtgaggcaacgttcaccactttggttccgggagcattcgcagatgaggcaccacacttcaaggttggtgtgttcgcccgtggcatgctggagcgtctgtacactcgcgcatacctgccagacgccgatttgagcaccgacccagttttggctgtggtcccagctgatcgacgtgacctcctggtggctcaaaagaccgatgatggattccgcttcgacatcactgtccaggctgaagacaatgaaaccccattttttggactctaa

SEQ ID NO: 34 - protein, 204 aa, Corynebacterium glutamicum
MIDTGKNGEFRYEQSNIIDQNEAEFGITPSQTVGPYVHIGLTLEGAEHLVEPGSEGAVSFTVSATDGNGDPIADAMFELWQADPEGIHNSDLDPNRTAPATADGFRGLGRAMANAQGEATFTTLVPGAFADEAPHFKVGVFARGMLERLYTRAYLPDADLSTDPVLAVVPADRRDLLVAQKTDDGFRFDITVQAEDNETPFFGL

SEQ ID NO: 35 - DNA, 693 bp, Corynebacterium glutamicum
atggacatcccacacttcgccccgacgggaggcgaatactccccactgcacttcccggagtaccggaccaccatcaagcgcaacccaagcaacgatctcatcatggttcctagtcgcctcggcgagtccacgggacctgtcttcggcgaccgcgacttgggagacatcgacaacgacatgaccaaggtgaacggtggcgaggctatcggccagcgcatcttcgttcacggccgtgtcctcggtttcgatggcaagccagttccgcacaccttggtcgaggcgtggcaggcaaacgccgcaggccgttaccgccacaagaatgactcctggccagcgccactggatccacacttcaacggtgttgcacgtactctcaccgacaaggacggccagtaccacttctggaccgttatgccaggtaattacccttggggtaaccaccacaacgcatggcgcccggcgcacattcacttctcgctctatggtcgtcagtttacggagcgtctggtcacccagatgtacttcccgaacgatccattgttcttccaggatccgatctacaacgcggtgccaaagggtgcacgtgagcgcatgatcgcaacgttcgactatgacgagacccgtgaaaacttcgcgcttggttacaagttcgacatcgtccttcgtggccgcaacgccaccccatttgagtaa

SEQ ID NO: 36 - protein, 230 aa, Corynebacterium glutamicum
MDIPHFAPTGGEYSPLHFPEYRTTIKRNPSNDLIMVPSRLGESTGPVFGDRDLGDIDNDMTKVNGGEAIGQRIFVHGRVLGFDGKPVPHTLVEAWQANAAGRYRHKNDSWPAPLDPHFNGVARTLTDKDGQYHFWTVMPGNYPWGNHHNAWRPAHIHFSLYGRQFTERLVTQMYFPNDPLFFQDPIYNAVPKGARERMIATFDYDETRENFALGYKFDIVLRGRNATPFE

SEQ ID NO: 37 - DNA, 1164 bp, Escherichia coli
atgaacaactttaatctgcacaccccaacccgcattctgtttggtaaaggcgcaatcgctggtttacgcgaacaaattcctcacgatgctcgcgtattgattacctacggcggcggcagcgtgaaaaaaaccggcgttctcgatcaagttctggatgccctgaaaggcatggacgtgctggaatttggcggtattgagccaaacccggcttatgaaacgctgatgaacgccgtgaaactggttcgcgaacagaaagtgactttcctgctggcggttggcggcggttctgtactggacggcaccaaatttatcgccgcagcggctaactatccggaaaatatcgatccgtggcacattctgcaaacgggcggtaaagagattaaaagcgccatcccgatgggctgtgtgctgacgctgccagcaaccggttcagaatccaacgcaggcgcggtgatctcccgtaaaaccacaggcgacaagcaggcgttccattctgcccatgttcagccggtatttgccgtgctcgatccggtttatacctacaccctgccgccgcgtcaggtggctaacggcgtagtggacgcctttgtacacaccgtggaacagtatgttaccaaaccggttgatgccaaaattcaggaccgtttcgcagaaggcattttgctgacgctaatcgaagatggtccgaaagccctgaaagagccagaaaactacgatgtgcgcgccaacgtcatgtgggcggcgactcaggcgctgaacggtttgattggcgctggcgtaccgcaggactgggcaacgcatatgctgggccacgaactgactgcgatgcacggtctggatcacgcgcaaacactggctatcgtcctgcctgcactgtggaatgaaaaacgcgataccaagcgcgctaagctgctgcaatatgctgaacgcgtctggaacatcactgaaggttccgatgatgagcgtattgacgccgcgattgccgcaacccgcaatttctttgagcaattaggcgtgccgacccacctctccgactacggtctggacggcagctccatcccggctttgctgaaaaaactggaagagcacggcatgacccaactgggcgaaaatcatgacattacgttggatgtcagccgccgtatatacgaagccgcccgctaa

SEQ ID NO: 38 - protein, 387 aa, Escherichia coli
MNNFNLHTPTRILFGKGAIAGLREQIPHDARVLITYGGGSVKKTGVLDQVLDALKGMDVLEFGGIEPNPAYETLMNAVKLVREQKVTFLLAVGGGSVLDGTKFIAAAANYPENIDPWHILQTGGKEIKSAIPMGCVLTLPATGSESNAGAVISRKTTGDKQAFHSAHVQPVFAVLDPVYTYTLPPRQVANGVVDAFVHTVEQYVTKPVDAKIQDRFAEGILLTLIEDGPKALKEPENYDVRANVMWAATQALNGLIGAGVPQDWATHMLGHELTAMHGLDHAQTLAIVLPALWNEKRDTKRAKLLQYAERVWNITEGSDDERIDAAIAATRNFFEQLGVPTHLSDYGLDGSSIPALLKKLEEHGMTQLGENHDITLDVSRRIYEAAR

SEQ ID NO: 39 - DNA, 1062 bp, Corynebacterium glutamicum
atgagcatccaagtaaaagcactccagaaaaccggccccgaagcacctttcgaggtcaaaatcattgagcgtcgtgagcctcgcgctgacgacgtagttatcgacatcaaagctgccggcatctgccacagcgatatccacaccatccgcaacgaatggggcgaggcacacttcccgctcaccgtcggccacgaaatcgcaggcgttgtctctgcggttggctccgatgtaaccaagtggaaagtcggcgaccgcgttggcgtcggctgcctagttaactcctgcggcgaatgtgaacagtgtgtcgcgggatttgaaaacaactgccttcgcggaaacgtcggaacctacaactccgacgacgtcgacggcaccatcacgcaaggtggctacgccgaaaaggtagtggtcaacgaacgtttcctctgcagcatcccagaggaactcgacttcgatgtcgcagcaccactgctgtgcgcaggcatcaccacctactccccgatcgctcgctggaacgttaaagaaggcgacaaagtagcagtcatgggcctcggcgggctcggccacatgggtgtccaaatcgccgcagccaagggcgctgacgttaccgttctgtcccgttccctgcgcaaggctgaacttgccaaggaactcggcgcagctcgcacgcttgcgacttctgatgaggatttcttcaccgaacacgccggtgaattcgacttcatcctcaacaccattagcgcatccatcccagtcgacaagtacctgagccttctcaagccacacggtgtcatggctgttgtcggtctgccaccagagaagcagccactgagcttcggtgcgctcatcggcggcggaaaagtcctcaccggatccaacattggcggcatccctgaaacccaggaaatgctcgacttctgtgcaaaacacggcctcggcgcgatgatcgaaactgtcggcgtcaacgatgttgatgcagcctacgaccgcgttgttgccggcgacgttcagttccgcgttgtcattgatactgcttcgtttgcagaggtagaggcggtttag

SEQ ID NO: 40 - protein, 353 aa, Corynebacterium glutamicum
MSIQVKALQKTGPEAPFEVKIIERREPRADDVVIDIKAAGICHSDIHTIRNEWGEAHFPLTVGHEIAGVVSAVGSDVTKWKVGDRVGVGCLVNSCGECEQCVAGFENNCLRGNVGTYNSDDVDGTITQGGYAEKVVVNERFLCSIPEELDFDVAAPLLCAGITTYSPIARWNVKEGDKVAVMGLGGLGHMGVQIAAAKGADVTVLSRSLRKAELAKELGAARTLATSDEDFFTEHAGEFDFILNTISASIPVDKYLSLLKPHGVMAVVGLPPEKQPLSFGALIGGGKVLTGSNIGGIPETQEMLDFCAKHGLGAMIETVGVNDVDAAYDRVVAGDVQFRVVIDTASFAEVEAV

SEQ ID NO: 41 - DNA, 1113 bp, Corynebacterium glutamicum
gtgtccatgagcactgtcgtgcctggaattgtcgccctgtccaagggggcaccggtagaaaaagtaaacgttgttgtccctgatccaggtgctaacgatgtcatcgtcaagattcaggcctgcggtgtgtgccacaccgacttggcctaccgcgatggcgatatttcagatgagttcccttacctcctcggccacgaggcagcaggtattgttgaggaggtaggcgagtccgtcacccacgttgaggtcggcgatttcgtcatcttgaactggcgtgcagtgtgcggcgagtgccgtgcatgtaagaagggcgagccaaagtactgctttaacacccacaacgcatctaagaagatgaccctggaagacggcaccgagctgtccccagcactgggtattggcgcgttcttggaaaagaccctggtccacgaaggccagtgcaccaaggttaaccctgaggaagatccagcagcagctggccttctgggttgcggcatcatggcaggtcttggtgctgcggtaaacaccggtgatattaagcgcggcgagtccgtggcagtcttcggccttggtggcgtgggcatggcagctattgctggcgccaagattgctggtgcatcgaagattattgctgttgatatcgatgagaagaagttggagtgggcgaaggaattcggcgcaacccacaccattaattcctctggtcttggtggcgagggtgatgcctctgaggtcgtggcaaaggttcgtgagctcactgatggtttcggtactgacgtctccatcgatgcggtaggcatcatgccgacctggcagcaggcgttttactcccgtgatcatgcaggccgcatggtgatggtgggcgttccaaacctgacgtctcgcgtagatgttcctgcgattgatttttacggtcgcggtggctctgtgcgccctgcatggtacggcgactgcctgcctgagcgtgatttcccaacttatgtggatctgcacctgcagggtcgtttcccgctggataagtttgtttctgagcgtattggtcttgatgatgttgaagaggctttcaacaccatgaaggctggcgacgtgctgcgttctgtggtggagatctaa

SEQ ID NO: 42 - protein, 370 aa, Corynebacterium glutamicum
MSMSTVVPGIVALSKGAPVEKVNVVVPDPGANDVIVKIQACGVCHTDLAYRDGDISDEFPYLLGHEAAGIVEEVGESVTHVEVGDFVILNWRAVCGECRACKKGEPKYCFNTHNASKKMTLEDGTELSPALGIGAFLEKTLVHEGQCTKVNPEEDPAAAGLLGCGIMAGLGAAVNTGDIKRGESVAVFGLGGVGMAAIAGAKIAGASKIIAVDIDEKKLEWAKEFGATHTINSSGLGGEGDASEVVAKVRELTDGFGTDVSIDAVGIMPTWQQAFYSRDHAGRMVMVGVPNLTSRVDVPAIDFYGRGGSVRPAWYGDCLPERDFPTYVDLHLQGRFPLDKFVSERIGLDDVEEAFNTMKAGDVLRSVVEI

SEQ ID NO: 43 - DNA, 1047 bp, Corynebacterium glutamicum
gtgagttttatgaccactgctgcaccccaagaatttaccgctgctgttgttgaaaaattcggtcatgacgtgaccgtgaaggatattgaccttccaaagccagggccacaccaggcattggtgaaggtactcacctccggcatctgccacaccgacctccacgccttggagggcgattggccagtaaagccggaaccaccattcgtaccaggacacgaaggtgtaggtgaagttgttgagctcggaccaggtgaacacgatgtgaaggtcggcgatattgtcggcaatgcgtggctctggtcagcgtgcggcacctgcgaatactgcatcacaggcagggaaactcagtgtaacgaagctgagtacggtggctacacccaaaatggatccttcggccagtacatgctggtggatacccgatacgccgctcgcatcccagacggcgtggactacctcgaagcagcgccaattctgtgtgcaggcgtgactgtctacaaggcactcaaagtctctgaaacccgcccgggccaattcatggtgatctccggtgtcggcggacttggccacatcgcagtccaatacgcagcggcgatgggcatgcgtgtcattgcggtagatattgccgaggacaagctggaacttgcccgtaagcacggtgcggaatttaccgtgaatgcgcgtaatgaagatccaggcgaagctgtacagaagtacaccaacggtggcgcacacggcgtgcttgtgactgcagttcacgaggcagcattcggccaggcactggatatggctcgacgtgcaggaacaattgtgttcaacggtctgccaccgggagagttcccagcatccgtgttcaacatcgtattcaagggcctgaccatccgtggatccctcgtgggaacccgccaagacttggccgaagcgctcgatttctttgcacgcggactaatcaagccaaccgtgagtgagtgctccctcgatgaggtcaatggagttcttgaccgcatgcgaaacggcaagatcgatggtcgtgtggcgattcgtttctaa

SEQ ID NO: 44 - protein, 348 aa, Corynebacterium glutamicum
MSFMTTAAPQEFTAAVVEKFGHDVTVKDIDLPKPGPHQALVKVLTSGICHTDLHALEGDWPVKPEPPFVPGHEGVGEVVELGPGEHDVKVGDIVGNAWLWSACGTCEYCITGRETQCNEAEYGGYTQNGSFGQYMLVDTRYAARIPDGVDYLEAAPILCAGVTVYKALKVSETRPGQFMVISGVGGLGHIAVQYAAAMGMRVIAVDIAEDKLELARKHGAEFTVNARNEDPGEAVQKYTNGGAHGVLVTAVHEAAFGQALDMARRAGTIVFNGLPPGEFPASVFNIVFKGLTIRGSLVGTRQDLAEALDFFARGLIKPTVSECSLDEVNGVLDRMRNGKIDGRVAIRF

SEQ ID NO: 45 - DNA, 1020 bp, Corynebacterium glutamicum
atgcccaaatacattgccatgcaggtatccgaatccggtgcaccgttagccgcgaatctcgtgcaacctgctccgttgaaatcgagggaagtccgcgtggaaatcgctgctagtggtgtgtgccatgcagatattggcacggcagcagcatcggggaagcacactgtttttcctgttacccctggtcatgagattgcaggaaccatcgcggaaattggtgaaaacgtatctcggtggacggttggtgatcgcgttgcaatcggttggtttggtggcaattgcggtgactgcgctttttgtcgtgcaggtgatcctgtgcattgcagagagcggaagattcctggcgtttcttatgcgggtggttgggcacagaatattgttgttccagcggaggctcttgctgcgattccagatggcatggacttttacgaggccgccccgatgggctgcgcaggtgtgacaacattcaatgcgttgcgaaacctgaagctggatcccggtgcggctgtcgcggtctttggaatcggcggtttagtgcgcctagctattcagtttgctgcgaaaatgggttatcgaaccatcaccatcgcccgcggtttagagcgtgaggagctagctaggcaacttggcgccaaccactacatcgatagcaatgatctgcaccctggccaggcgttatttgaacttggcggggctgacttgatcttgtctactgcgtccaccacggagcctctttcggagttgtctaccggtctttctattggcgggcagctaaccattatcggagttgatgggggagatatcaccgtttcggcagcccaattgatgatgaaccgtcagatcatcacaggtcacctcactggaagtgcgaatgacacggaacagactatgaaatttgctcatctccatggcgtgaaaccgcttattgaacggatgcctctcgatcaagccaacgaggctattgcacgtatttcagctggtaaaccacgtttccgtattgtcttggagccgaattcataa

SEQ ID NO: 46 - protein, 339 aa, Corynebacterium glutamicum
MPKYIAMQVSESGAPLAANLVQPAPLKSREVRVEIAASGVCHADIGTAAASGKHTVFPVTPGHEIAGTIAEIGENVSRWTVGDRVAIGWFGGNCGDCAFCRAGDPVHCRERKIPGVSYAGGWAQNIVVPAEALAAIPDGMDFYEAAPMGCAGVTTFNALRNLKLDPGAAVAVFGIGGLVRLAIQFAAKMGYRTITIARGLEREELARQLGANHYIDSNDLHPGQALFELGGADLILSTASTTEPLSELSTGLSIGGQLTIIGVDGGDITVSAAQLMMNRQIITGHLTGSANDTEQTMKFAHLHGVKPLIERMPLDQANEAIARISAGKPRFRIVLEPNS

SEQ ID NO: 47 - DNA, 879 bp, Corynebacterium glutamicum
atgcaaacccttgctgctattgttcgtgccacgaagcaaccttttgagatcaccaccattgatctggatgcaccacgaccagatgaagttcaaatccgtgttattgctgccggagtgcgccacactgacgcaattgttcgtgatcagatttacccaacttttcttcccgcagttttcggccacgaaggcgccggagtagttgtcgccgtgggttctgcagtcacctcggtgaaaccagatgacaaggtagtgctgggattcaactcttgtggccagtgcttgaagtgtttgggcggtaagcctgcgtactgtgagaaattctatgaccgcaacttcgcatgcacccgcgatgccgggcacactactttgtttacccgtgcaacaaaagagcaggcagaggccatcatcgacacccttgatgatgttttctacgatgcggatgcgggtttcctggcatacccagcaactcccccagaggcttcgggagtaagcgtgttggttgtcgcggctggtacctctgatctcccccaagcaaaggaagcactacacactgcctcctacttggggcgctccacctcactgattgttgattttggagtggctggcatccaccgcctgctttcatacgaagaagaactccgcgctgcgggcgtgctcatcgttgccgctggaatggatggtgcgctacccggagttgtcgcaggcttagtgtccgcacctgtcgtcgcactgccaacctccgtgggatacggcgcaggtgctggaggaatcgcaccacttctgaccatgcttaacgcctgcgcgccgggagttggagtggtcaacattgataacggctatggagcaggacacctggctgcgcagattgcggcgaggtaa

SEQ ID NO: 48 - protein, 292 aa, Corynebacterium glutamicum
MQTLAAIVRATKQPFEITTIDLDAPRPDEVQIRVIAAGVRHTDAIVRDQIYPTFLPAVFGHEGAGVVVAVGSAVTSVKPDDKVVLGFNSCGQCLKCLGGKPAYCEKFYDRNFACTRDAGHTTLFTRATKEQAEAIIDTLDDVFYDADAGFLAYPATPPEASGVSVLVVAAGTSDLPQAKEALHTASYLGRSTSLIVDFGVAGIHRLLSYEEELRAAGVLIVAAGMDGALPGVVAGLVSAPVVALPTSVGYGAGAGGIAPLLTMLNACAPGVGVVNIDNGYGAGHLAAQIAAR

SEQ ID NO: 49 - DNA, 819 bp, Escherichia coli
atggaaacctatgctgtttttggtaatccgatagcccacagcaaatcgccattcattcatcagcaatttgctcagcaactgaatattgaacatccctatgggcgcgtgttggcacccatcaatgatttcatcaacacactgaacgctttctttagtgctggtggtaaaggtgcgaatgtgacggtgccttttaaagaagaggcttttgccagagcggatgagcttactgaacgggcagcgttggctggtgctgttaataccctcatgcggttagaagatggacgcctgctgggtgacaataccgatggtgtaggcttgttaagcgatctggaacgtctgtcttttatccgccctggtttacgtattctgcttatcggcgctggtggagcatctcgcggcgtactactgccactcctttccctggactgtgcggtgacaataactaatcggacggtatcccgcgcggaagagttggctaaattgtttgcgcacactggcagtattcaggcgttgagtatggacgaactggaaggtcatgagtttgatctcattattaatgcaacatccagtggcatcagtggtgatattccggcgatcccgtcatcgctcattcatccaggcatttattgctatgacatgttctatcagaaaggaaaaactccttttctggcatggtgtgagcagcgaggctcaaagcgtaatgctgatggtttaggaatgctggtggcacaggcggctcatgcctttcttctctggcacggtgttctgcctgacgtagaaccagttataaagcaattgcaggaggaattgtccgcgtga

SEQ ID NO: 50 - protein, 272 aa, Escherichia coli
METYAVFGNPIAHSKSPFIHQQFAQQLNIEHPYGRVLAPINDFINTLNAFFSAGGKGANVTVPFKEEAFARADELTERAALAGAVNTLMRLEDGRLLGDNTDGVGLLSDLERLSFIRPGLRILLIGAGGASRGVLLPLLSLDCAVTITNRTVSRAEELAKLFAHTGSIQALSMDELEGHEFDLIINATSSGISGDIPAIPSSLIHPGIYCYDMFYQKGKTPFLAWCEQRGSKRNADGLGMLVAQAAHAFLLWHGVLPDVEPVIKQLQEELSA

SEQ ID NO: 51 - DNA, 35 bp, Artificial Sequence
  primer
cggtacccggggatccttacttccgcgtatccaac

SEQ ID NO: 52 - DNA, 41 bp, Artificial Sequence
  primer
ctaggaatcgcggccggtgaactcctaaagaactatataac

SEQ ID NO: 53 - DNA, 20 bp, Artificial Sequence
  primer
ggccgcgattcctagcatgc

SEQ ID NO: 54 - DNA, 35 bp, Artificial Sequence
  primer
ccaagcttgcatgccagtcatcatcaacggtgccg

SEQ ID NO: 55 - DNA, 21 bp, Artificial Sequence
  primer
atctccgcagaagacgtactg

SEQ ID NO: 56 - DNA, 20 bp, Artificial Sequence
  primer
tccgatcatgtatgacctcc

SEQ ID NO: 57 - DNA, 36 bp, Artificial Sequence
  primer
cggtacccggggatcggcatagtgcttccaacgctc

SEQ ID NO: 58 - DNA, 36 bp, Artificial Sequence
  primer
tagctccactcaagattcctcgatattacctacagg

SEQ ID NO: 59 - DNA, 20 bp, Artificial Sequence
  primer
tcttgagtggagctagggcc

SEQ ID NO: 60 - DNA, 37 bp, Artificial Sequence
  primer
ccaagcttgcatgcccatatagagcccaggagctctc

SEQ ID NO: 61 - DNA, 23 bp, Artificial Sequence
  primer
cgccgcaaagtccaaatagaaag

SEQ ID NO: 62 - DNA, 20 bp, Artificial Sequence
  primer
ggattcttcctgaactcagc

SEQ ID NO: 63 - DNA, 36 bp, Artificial Sequence
  primer
cggtacccggggatcgggctcgtcctgaaattgcac

SEQ ID NO: 64 - DNA, 35 bp, Artificial Sequence
  primer
tccgtcgtgagccatgttgtgcccacgagactacc

SEQ ID NO: 65 - DNA, 20 bp, Artificial Sequence
  primer
atggctcacgacggattgcg

SEQ ID NO: 66 - DNA, 36 bp, Artificial Sequence
  primer
ccaagcttgcatgcccggttgcagccttcataaacg

SEQ ID NO: 67 - DNA, 21 bp, Artificial Sequence
  primer
agaccaatgagtacccaaccg

SEQ ID NO: 68 - DNA, 20 bp, Artificial Sequence
  primer
tcagcgtctggctcagctac

SEQ ID NO: 69 - DNA, 36 bp, Artificial Sequence
  primer
cggtacccggggatcaaccccagctcaaataacacc

SEQ ID NO: 70 - DNA, 37 bp, Artificial Sequence
  primer
tttcaacacaatccgtccttctcgcttggattacttg

SEQ ID NO: 71 - DNA, 23 bp, Artificial Sequence
  primer
cggattgtgttgaaattgctctg

SEQ ID NO: 72 - DNA, 35 bp, Artificial Sequence
  primer
ccaagcttgcatgcctcaccacgggaatcttcagg

SEQ ID NO: 73 - DNA, 20 bp, Artificial Sequence
  primer
ccggactggggtgtgttttg

SEQ ID NO: 74 - DNA, 20 bp, Artificial Sequence
  primer
cccggaaaatacggtatagc

SEQ ID NO: 75 - DNA, 35 bp, Artificial Sequence
  primer
ccaagcttgcatgccccatcgcattgccgaaaagc

SEQ ID NO: 76 - DNA, 35 bp, Artificial Sequence
  primer
aaagatcgggtcaatgcagttcgcggggcgaacat

SEQ ID NO: 77 - DNA, 35 bp, Artificial Sequence
  primer
cgccccgcgaactgcattgacccgatctttatacc

SEQ ID NO: 78 - DNA, 35 bp, Artificial Sequence
  primer
cggtacccggggatcaacgttgacggtgatgccat

SEQ ID NO: 79 - DNA, 25 bp, Artificial Sequence
  primer
gaaatgtcatacttcagccatcagg

SEQ ID NO: 80 - DNA, 25 bp, Artificial Sequence
  primer
tgcgagtgatgaaatcctgaaactt

SEQ ID NO: 81 - DNA, 35 bp, Artificial Sequence
  primer
ccaagcttgcatgcctttcgcggtgaatcaaccca

SEQ ID NO: 82 - DNA, 35 bp, Artificial Sequence
  primer
caggtcaaagctaaggcattgtctgtaaatgggca

SEQ ID NO: 83 - DNA, 35 bp, Artificial Sequence
  primer
ctaaggggtttagcaatgcccaatcaggcccactt

SEQ ID NO: 84 - DNA, 35 bp, Artificial Sequence
  primer
cggtacccggggatcttagggtacgagggtaagtg

SEQ ID NO: 85 - DNA, 93 bp, Artificial Sequence
  DNA fragment of P2 promoter
cttagctttgacctgcacaaatagttgcaaattgtcccacatacacataaagtagcttgcgtatttaaaattatgaacctaaggggtttagca

SEQ ID NO: 86 - DNA, 35 bp, Artificial Sequence
  primer
atttacagacaatgccttagctttgacctgcacaa

SEQ ID NO: 87 - DNA, 31 bp, Artificial Sequence
  primer
ggcctgattgggcattgctaaaccccttagg

SEQ ID NO: 88 - DNA, 1686 bp, Corynebacterium glutamicum
atgacaacaaccaccggaagtgcccggccagcacgtgccgccaggaagcctaagcccgaaggccaatggaaaatcgacggcaccgagccgcttaaccatgccgaggaaattaagcaagaagaacccgcttttgctgtcaagcagcgggtcattgatatttactccaagcagggtttttcttccattgcaccggatgacattgccccacgctttaagtggttgggcatttacacccagcgtaagcaggatctgggcggtgaactgaccggtcagcttcctgatgatgagctgcaggatgagtacttcatgatgcgtgtgcgttttgatggcggactggcttcccctgagcgcctgcgtgccgtgggtgaaatttctagggattatgctcgttccaccgcggacttcaccgaccgccagaacattcagctgcactggattcgtattgaagatgtgcctgcgatctgggagaagctagaaaccgtcggactgtccaccatgcttggttgcggtgacgttccacgtgttatcttgggctccccagtttctggcgtagctgctgaagagctgatcgatgccaccccggctatcgatgcgattcgtgagcgctacctagacaaggaagagttccacaaccttcctcgtaagtttaagactgctatcactggcaaccagcgccaggatgttacccacgaaatccaggacgtttccttcgttccttcgattcacccagaattcggcccaggatttgagtgctttgtgggcggcggcctgtccaccaacccaatgcttgctcagccacttggttcttggattccacttgatgaggttccagaagtgtgggctggcgtcgccggaattttccgcgactacggcttccgacgcctgcgtaaccgtgctcgcctcaagttcttggtggcacagtggggtattgagaagttccgtgaagttcttgagaccgaatacctcgagcgcaagctgattgatggcccagttgttaccaccaaccctggctaccgtgaccacattggcattcacccacaaaaggacggcaagttctacctcggtgtgaagccaaccgttggacacaccaccggtgagcagctcattgccattgctgatgttgcagaaaagcacggcatcaccaggattcgtaccacggcggaaaaggaactgctcttcctcgatattgagcgagagaaccttactaccgttgcacgtgacctggatgaaatcggactgtactcttcaccttccgagttccgccgcggcatcatttcctgcaccggcttggagttctgcaagcttgcgcacgcaaccaccaagtcacgagcaattgagcttgtggacgaactggaagagcgactcggcgatttggatgttcccatcaagattgccctgaacggttgccctaactcttgtgcacgcacccaggtttccgacatcggattcaagggacagaccgtcactgatgctgacggcaaccgcgttgaaggtttccaggttcacctgggcggttccatgaacttggatccaaacttcggacgcaagctcaagggccacaaggttattgccgatgaagtgggagagtacgtcactcgcgttgttacccacttcaaggaacagcgccacgaggacgagcacttccgcgattgggtccagcgggccgctgaggaagatttggtgtga

SEQ ID NO: 89 - protein, 561 aa, Corynebacterium glutamicum
MTTTTGSARPARAARKPKPEGQWKIDGTEPLNHAEEIKQEEPAFAVKQRVIDIYSKQGFSSIAPDDIAPRFKWLGIYTQRKQDLGGELTGQLPDDELQDEYFMMRVRFDGGLASPERLRAVGEISRDYARSTADFTDRQNIQLHWIRIEDVPAIWEKLETVGLSTMLGCGDVPRVILGSPVSGVAAEELIDATPAIDAIRERYLDKEEFHNLPRKFKTAITGNQRQDVTHEIQDVSFVPSIHPEFGPGFECFVGGGLSTNPMLAQPLGSWIPLDEVPEVWAGVAGIFRDYGFRRLRNRARLKFLVAQWGIEKFREVLETEYLERKLIDGPVVTTNPGYRDHIGIHPQKDGKFYLGVKPTVGHTTGEQLIAIADVAEKHGITRIRTTAEKELLFLDIERENLTTVARDLDEIGLYSSPSEFRRGIISCTGLEFCKLAHATTKSRAIELVDELEERLGDLDVPIKIALNGCPNSCARTQVSDIGFKGQTVTDADGNRVEGFQVHLGGSMNLDPNFGRKLKGHKVIADEVGEYVTRVVTHFKEQRHEDEHFRDWVQRAAEEDLV

SEQ ID NO: 90 - DNA, 249 bp, Corynebacterium glutamicum
gtgagtcttcggaggaaacccaatcccaaccgcaaccaccctctgtactgcccatactgcgcgggagaagttcttttccccgatgagcaaacagaattcgcgtggttgtgtgcggattgcaccagagtttttgaagtgaaatatcacggccaggacgatccagtgcacaggccagcaccagcaaagtccacatcgcaagcattaaaagaatctctcgaaagacacaaaagaggtgagtcgcaacaatga

SEQ ID NO: 91 - protein, 82 aa, Corynebacterium glutamicum
MSLRRKPNPNRNHPLYCPYCAGEVLFPDEQTEFAWLCADCTRVFEVKYHGQDDPVHRPAPAKSTSQALKESLERHKRGESQQ

SEQ ID NO: 92 - DNA, 786 bp, Corynebacterium glutamicum
atgagctttcaactagttaacgccctgaaaaatactggttcggtaaaagatcccgagatctcacccgaaggacctcgcacgaccacaccgttgtcaccagaggtagcaaaacacaacgaggaactcgtcgaaaagcatgctgctgcgttgtatgacgccagcgcgcaagagatcctggaatggacagccgagcacacgccgggcgctattgcagtgaccttgagcatggaaaacaccgtgctggcggagctggctgcgcggcacctgccggaagctgatttcctctttttggacaccggttaccacttcaaggaaactcttgaagttgcccgccaggtagatgagcgttattcccagaagcttgtcaccgcgctgccaatcctcaagcgcacggagcaggattccatttatggtctcaacctgtaccgcagcaacccagcggcgtgctgccgaatgcgcaaagttgaaccgctggcggcgtcgttaagcccatacgctggctggatcaccggcctgcgccgcgctgatggcccaacccgtgctcaagcccctgcgctgagcttggatgccaccggcaggctcaagatttctccaattatcacctggtcattggaggaaaccaacgagttcattgcggacaacaacctcatcgatcacccacttacccatcagggttatccatcaattggatgcgaaacctgcacccttcctgttgctgaaggacaagaccctagggccggccgttgggctggaaacgccaagacagaatgcggacttcactcatga

SEQ ID NO: 93 - protein, 261 aa, Corynebacterium glutamicum
MSFQLVNALKNTGSVKDPEISPEGPRTTTPLSPEVAKHNEELVEKHAAALYDASAQEILEWTAEHTPGAIAVTLSMENTVLAELAARHLPEADFLFLDTGYHFKETLEVARQVDERYSQKLVTALPILKRTEQDSIYGLNLYRSNPAACCRMRKVEPLAASLSPYAGWITGLRRADGPTRAQAPALSLDATGRLKISPIITWSLEETNEFIADNNLIDHPLTHQGYPSIGCETCTLPVAEGQDPRAGRWAGNAKTECGLHS

SEQ ID NO: 94 - DNA, 954 bp, Corynebacterium glutamicum
ttgggctggaaacgccaagacagaatgcggacttcactcatgaccacaaccgttgcatcagaactttccccacaccttaaagatcttgaaaatgaatccatccacatcctccgcgaggtagctggccagtttgataaggtcggcctgctgttttccggcggtaaggattccgtcgtggtgtacgagcttgcgcgccgcgctttcgctccagctaacgtgccttttgaattgctgcacgtggacaccggccacaacttcccagaggttttggaattccgcgacaacctggtggagcgcaccggcgcccgcctgcgcgtagctaaagtccaggactggatcgatcgcggtgacctgcaggaacgcccagacggcacccgcaacccactgcagactgtccctttggtggagaccatcgctgagcagggctacgacgccgtgcttggtggcgctcgccgcgatgaggagcgtgcccgcgccaaggagcgtgtgttctctgtgcgtgactccttcggtggttgggatccacgccgtcagcgcccagagctgtggaccctctacaacggtggccacctgccaggcgaaaacatccgtgttttcccaatctccaactggactgaagctgacatctgggagtacatcggcgcccgtggcatcgaacttccaccgatctacttctcccacgaccgcgaagttttcgagcgcgacggcatgtggctgaccgcaggcgagtggggtggaccaaagaagggcgaggagatcgtcaccaagactgtccgctaccgcaccgtcggcgatatgtcctgcaccggtgctgtgctctcagaagcccgcaccattgacgatgtgatcgaagagatcgccacctccacccttaccgaacgtggcgcaacccgcgccgatgaccgcctcagcgaatccgcaatggaagaccgcaagaaggaaggctacttctga

SEQ ID NO: 95 - protein, 317 aa, Corynebacterium glutamicum
MGWKRQDRMRTSLMTTTVASELSPHLKDLENESIHILREVAGQFDKVGLLFSGGKDSVVVYELARRAFAPANVPFELLHVDTGHNFPEVLEFRDNLVERTGARLRVAKVQDWIDRGDLQERPDGTRNPLQTVPLVETIAEQGYDAVLGGARRDEERARAKERVFSVRDSFGGWDPRRQRPELWTLYNGGHLPGENIRVFPISNWTEADIWEYIGARGIELPPIYFSHDREVFERDGMWLTAGEWGGPKKGEEIVTKTVRYRTVGDMSCTGAVLSEARTIDDVIEEIATSTLTERGATRADDRLSESAMEDRKKEGYF

SEQ ID NO: 96 - DNA, 1302 bp, Corynebacterium glutamicum
atgactgctccaaccttgaataaagcatccgaaaagattgcatcacgcgagacccttcgtctgtgcaccgcaggttccgtagatgatggcaagtccaccttcgtcggccgcctcctgcacgacaccaagtctgttcttgctgatcagctagcttccgtagagcgcacctccgccgaccgcggcttcgaaggcctcgacctgtccctcctcgtcgacggcctgcgcgccgagcgtgagcagggcatcaccatcgacgttgcctaccgctacttcgccactgacaagcgcaccttcatcctggctgacaccccaggccacgtgcagtacacccgcaacaccgtcaccggcgtctccacctcccaggttgtagttttgcttgtcgacgcccgccacggcgtcgtcgagcagacccgccgccacctgtccgtatcggccctgctgggcgtgcgcacggtgatcctcgcagtcaacaaaattgaccttgttgattacagcgaagaagtcttccgcaacattgaaaaagaattcgtttctttggcttccgctttagatgtcaccgacacccacgtcgttccgatctccgcactcaagggcgacaacgttgcagaaccttccacccacatggactggtacgcgggaccaaccgtgctggaaatcctggaaaacgttgaagtttcccgcggccgtgcacacgacctgggcttccgcttcccaatccagtacgtcatccgcgagcacgcaaccgattaccgcggctacgccggcaccatcaacgctggttccatctccgtgggcgataccgtgcacctacctgaaggccgcaccacccaggtcacccacatcgattccgctgacggatccctccaaaccgcatcagttggagaagccgttgtcctgcgcctagcccaggaaatcgacctcatccgcggcgaactcatcgcaggctccgatcgcccagaatccgttcgttccttcaacgccactgtcgttggtctagcagatcgcactatcaaaccaggtgcagcagtcaaggtccgctacggcaccgagctggtccgcggacgcgtcgcagccatcgaacgagtcctcgacatcgacggcgtcaacgacaacgaagcaccagaaacctacggcctcaacgacatcgcgcacgtgcgcatcgatgttgcaggtgaattggaagttgaagattacgctgctcgtggcgcaattggctccttccttcttatcgatcaatcctccggcgacaccctcgctgccggtttggttggccaccgcctacgcaataactggtcgatctag

SEQ ID NO: 97 - protein, 433 aa, Corynebacterium glutamicum
MTAPTLNKASEKIASRETLRLCTAGSVDDGKSTFVGRLLHDTKSVLADQLASVERTSADRGFEGLDLSLLVDGLRAEREQGITIDVAYRYFATDKRTFILADTPGHVQYTRNTVTGVSTSQVVVLLVDARHGVVEQTRRHLSVSALLGVRTVILAVNKIDLVDYSEEVFRNIEKEFVSLASALDVTDTHVVPISALKGDNVAEPSTHMDWYAGPTVLEILENVEVSRGRAHDLGFRFPIQYVIREHATDYRGYAGTINAGSISVGDTVHLPEGRTTQVTHIDSADGSLQTASVGEAVVLRLAQEIDLIRGELIAGSDRPESVRSFNATVVGLADRTIKPGAAVKVRYGTELVRGRVAAIERVLDIDGVNDNEAPETYGLNDIAHVRIDVAGELEVEDYAARGAIGSFLLIDQSSGDTLAAGLVGHRLRNNWSI

SEQ ID NO: 98 - DNA, 900 bp, Corynebacterium glutamicum
ttggctccttccttcttatcgatcaatcctccggcgacaccctcgctgccggtttggttggccaccgcctacgcaataactggtcgatctagaccagttgctgtgaaggcaaggtgccggcttagatgccggcgcctagcctacatccagctaagaccccctttaggacacctcatgattcccctgattacgctttcccacggttcccgcaaaaagtccgcagctgcaggtattactgcgctgactcatgaggccggacgaatgctggaaacaccagccgtggaagcgcatttagagcttgctgaaccttcccttgatcaggttgtggcaacgctcagtgcggaaggcgtaaccagggcagcgttggttcctttgctgtttagcaatgcgtatcacgcaaagattgacgttcctgaggcagtaaaagatgcttcagaaaagtatggtgtggaacttctcgtgggtccgcatttgggcactggctccgatgtagccagcgtgcttgcgcagcggttgcgtgcggacgcccccacagatgcccatgtgattttgtattccgttggcagctcacacgtgtccgccaatgaatcagtcatcgatcttgcccacaccattgctctcctcactggcttttcggttgaggtggtgcccgctaccggtgggccaggtgccggcggcgccggagtaatagaggtggcctcgaaacacaaggccgtccacatcctgccgctgtttgttacggaaggtttgctgctggatcgggttattgatcaatccgccaacatcgcagctgccaccggcacgaactttacctattccgaacccctaactactgacctcgcaccacttgttgcagcccgttaccacgctgcattgagcgcactgctggcacatatctaa

SEQ ID NO: 99 - protein, 299 aa, Corynebacterium glutamicum
MAPSFLSINPPATPSLPVWLATAYAITGRSRPVAVKARCRLRCRRLAYIQLRPPLGHLMIPLITLSHGSRKKSAAAGITALTHEAGRMLETPAVEAHLELAEPSLDQVVATLSAEGVTRAALVPLLFSNAYHAKIDVPEAVKDASEKYGVELLVGPHLGTGSDVASVLAQRLRADAPTDAHVILYSVGSSHVSANESVIDLAHTIALLTGFSVEVVPATGGPGAGGAGVIEVASKHKAVHILPLFVTEGLLLDRVIDQSANIAAATGTNFTYSEPLTTDLAPLVAARYHAALSALLAHI

SEQ ID NO: 100 - DNA, 930 bp, Corynebacterium glutamicum
atgcagacattaatctttatcgccattgcaggcgtcgcagcacagcttgttgatggcggcctcggcatggggttcggcgtcacctcaaccaccatcctcatcatgctcgcaggtttaggccctgcgcaggcatccgccgtcgtgcacaccgcagaggttggaaccaccttagtttctggtttaagccactggaaatttggcaacgtggattggaaagtagttgtccggctcggtatccccggcgctatcggcgcatttgctggcgctaccttcttgtccaatatttccaccgaagcagcagcaccgatcacctccctgattcttgccctgatcggcatgaacctagtctggcgattcagcaagggacgcatccgccgcgactattccgatcgcccgcacagcaagggattcctcggcggactcggtattgtcggtggcttcgttgacgcgtccggtggcggcggatggggtccagtgaccacctctacgctgctgtctttgggacgcaccgaaccccgcaaagtagtcggcaccgtcaacaccgcagaattcttagtctccctagccgcaacattgggcttcgtcgtgggactgtgggatgacctagtagctaacctctctgcagttctcgcgttgctcatcggcggcgcaatcgcagcaccaatcggcgcctggatgatctctcgcgttaatgcaaccgtcctcggcggcttcgtgggcaccctgattgtcacactgaacctgccaaaggtgctcaatgtggttggccttgatttcatccccaccggcctcgtccaggtcaccgtcctcctcatcggcctgccgctgacgtacctcggcttccgccgctaccgcaaaaacctcctcaacgaaaccatctccagcgaggttgtctccgaaccacagggacaaaagattaaaagctcttaa

SEQ ID NO: 101 - protein, 309 aa, Corynebacterium glutamicum
MQTLIFIAIAGVAAQLVDGGLGMGFGVTSTTILIMLAGLGPAQASAVVHTAEVGTTLVSGLSHWKFGNVDWKVVVRLGIPGAIGAFAGATFLSNISTEAAAPITSLILALIGMNLVWRFSKGRIRRDYSDRPHSKGFLGGLGIVGGFVDASGGGGWGPVTTSTLLSLGRTEPRKVVGTVNTAEFLVSLAATLGFVVGLWDDLVANLSAVLALLIGGAIAAPIGAWMISRVNATVLGGFVGTLIVTLNLPKVLNVVGLDFIPTGLVQVTVLLIGLPLTYLGFRRYRKNLLNETISSEVVSEPQGQKIKSS

SEQ ID NO: 102 - DNA, 1374 bp, Corynebacterium glutamicum
atgacaactcccctgcgcgtagccatcatcggagctggccctgctggcatttacgcatccgacctcctcatccgcaatgaagagcgcgaagtgttcgttgaccttttcgagcaaatgcctgcaccgttcggactcatccgttacggcgttgcaccagaccacccacgcatcaagggcatcgttaagtccctgcacaacgtgttggacaagccacgcctgcgcctgctcggcaacattgaaatcggcaaagacatcaccgtcgaagaactccgcgactactacgacgcagttgtcttctccaccggtgcagttgcagaccgcgacctcaacatccccggaattgaagcagaaggttccttcggtgccggcgagttcgttggcttctacgacggcaacccacgcttcgagcgctcctgggatctgtctgcacagtccgtcgctgttatcggcgttggtaacgtcggcctcgatgtagcccgcatcctggctaagacaggcgacgagctcaaagtcaccgaaatttccgacaacgtctacgactccctcaaagaaaacaaggccactgaagtacacgttttcggacgtcgtggcccagcacaggtcaagttcaccccacaggaactcaaagaactcgaccactcccccaccatcaacgtggttgttgacccagaagacatcgactacgacggcgcctccgaagaagcccgccgcgcatccaaatcccaggacctggtctgccagatcctggaacagtacgcaatccgcgagccaaaggacgctccgcacaccctgcagatccacctctttgaaaacccagttgaggttcttcaaaaggacggcaaggttgttggcctgcgcaccgaacgcaccgcgctcgacggcaacggtggcgtaaacggcaccggcgaattcaaggactggccagttcaggctgtctaccgcgcagtcggctacaagtccgaccccatcgacggcgtcccattcgatgggaacaagcacgtcatccctaatgacggcggacatgtcctcaccgctccaggtgcagagccagtaccaggcctctacgccaccggctggatcaagcgtggaccaatcggtctgatcggcaacaccaagtctgatgccaaggaaaccaccgacatcctcatcaaggatgccgtcaccggtgtacttgaagccccaaagcaccagggcgaagaagccatcatcgagcttctcgattcccgcaacatcccattcaccacctgggaaggctggtacaaactcgacgcagcagagcgcgcactcggtgaagccgaaggccgcgagcgcaagaagattgttgattgggaagaaatggtccgccaggcccgcgaagctccagcaattgtctaa

SEQ ID NO: 103 - protein, 457 aa, Corynebacterium glutamicum
MTTPLRVAIIGAGPAGIYASDLLIRNEEREVFVDLFEQMPAPFGLIRYGVAPDHPRIKGIVKSLHNVLDKPRLRLLGNIEIGKDITVEELRDYYDAVVFSTGAVADRDLNIPGIEAEGSFGAGEFVGFYDGNPRFERSWDLSAQSVAVIGVGNVGLDVARILAKTGDELKVTEISDNVYDSLKENKATEVHVFGRRGPAQVKFTPQELKELDHSPTINVVVDPEDIDYDGASEEARRASKSQDLVCQILEQYAIREPKDAPHTLQIHLFENPVEVLQKDGKVVGLRTERTALDGNGGVNGTGEFKDWPVQAVYRAVGYKSDPIDGVPFDGNKHVIPNDGGHVLTAPGAEPVPGLYATGWIKRGPIGLIGNTKSDAKETTDILIKDAVTGVLEAPKHQGEEAIIELLDSRNIPFTTWEGWYKLDAAERALGEAEGRERKKIVDWEEMVRQAREAPAIV

SEQ ID NO: 104 - DNA, 1173 bp, Corynebacterium glutamicum
ttgtctatgattggctatggtttacctatgcccaatcaggcccacttctctgcgtcctttgcccgcccctctaccccggctgcaaagtgcatgcaccatatccgcctcggccagcaactcattagaaatgagctggtcgaggccacaggtctgtcccaaccgactgtcacccgcgcagtcaccgctttaatgcaggcaggtttggttcgtgaacgccctgatctcacactctcatcgggccctggtcgtcccaatattcctctagaactcgctccaagtccatggattcatgcaggcgtggcaatcggcaccaagtcttcctacgtcgctttgtttgataccaagggtcgcacccttcgtgatgccatactggaaatctcagcagctgatttagatccagacaccttcatcgaacacctcatcgctggtgtcaaccgcctcaccactggtcttgatctaccactggtaggtattggtgtggctacctcaggaaaagtcaccaacgcgggcgttgtcaccgcaagcaacttgggctgggatggcgttgatatcgccggccgtctgaactaccaattcagcgttccagcaaccgtggcatcagcaattcctgccatcgcagcttctgaactgcaggcttccccacttccccaccctgagcagccaactcccatcaccttgaccttctacgccgatgactctgtgggcgcggcctacagcaatgatttgggagtacatgtcattggaccactggctacaactcgtggatcaggtttggatactttgggcatggctgctgaagatgcgctgagcacccaaggtttcttaagcagggtttctgatcagggtatctttgccaacagccttggtgagctagtcaccattgctaaagacaatgaaaccgcacgggaattcctcaacgatcgcgcgaccctgctggctcacactgccgcagaagctgctgaaacagttaagccatccaccctggttctctcgggatcggcgttttccgaagatccacaaggtcggttggtgttcgcttcccaattgaagaaggaatacgacgcagacattgagctccgcttgatccccacccaccgggaaaatgtccgcgcagcagctcgcgcagtcgcacttgatcgactactcaacgagccacttaccctcgtaccctaa

SEQ ID NO: 105 - protein, 390 aa, Corynebacterium glutamicum
LSMIGYGLPMPNQAHFSASFARPSTPAAKCMHHIRLGQQLIRNELVEATGLSQPTVTRAVTALMQAGLVRERPDLTLSSGPGRPNIPLELAPSPWIHAGVAIGTKSSYVALFDTKGRTLRDAILEISAADLDPDTFIEHLIAGVNRLTTGLDLPLVGIGVATSGKVTNAGVVTASNLGWDGVDIAGRLNYQFSVPATVASAIPAIAASELQASPLPHPEQPTPITLTFYADDSVGAAYSNDLGVHVIGPLATTRGSGLDTLGMAAEDALSTQGFLSRVSDQGIFANSLGELVTIAKDNETAREFLNDRATLLAHTAAEAAETVKPSTLVLSGSAFSEDPQGRLVFASQLKKEYDADIELRLIPTHRENVRAAARAVALDRLLNEPLTLVP

SEQ ID NO: 106 - DNA, 1074 bp, Corynebacterium glutamicum
gtgttcatgcttgcacagcgaacactccccattcacatcaccgccccccacctgcccgtcgcgcgcgtatttcaccaaattcgcgccacagacgccgatcgcacctcgctgcaacgcgatcttgaactctcccaagctggcatcactcggcatgtatcagcgcttattgatgcaggtctcgtggaggaaacccgagtggattccggggcgcgctcggggcgaccgcgcacaaaattaggcatcgacggccgccatctcaccgcctggggagtgcacattggcctgcgcagcacggattttgcggtgtgcgatttagccggccgagtgattaggtatgagcgcgtggaccatgaagtttcacactccacgccgtcggaaacgctgaattttgtcgcacataggttacaaacattgagcgccggcttgcccgagccccgcaatgtgggcgtggcattatctgcccacttaagcgccaacggcaccgtcacttccgaagattatggctggtcagaggtggaaattgggatacacctccccttccccgccaccatcggatcaggtgttgcggcgatggccggttcggaaattatcaacgcgccactgacccaatccacgcagtccacgctgtatttctacgcccgcgaaatggtctcccacgcctggattttcaacggcgctgtccaccgccccaacagcggccgcacgccgacggcgttcggaaatacaaataccttaaaagatgcttttcgacgtggactcacaccaacaactttctccgatttagtccaactctcccacaccaacccgcttgcccgacagatcctcaacgagcgcgcccacaaacttgccgacgccgtaaccaccgccgttgatgttgtcgaccccgaagccgtcgtcttcgccggcgaagccttcaccctggatccggaaactcttcgcattgtggtgacccagctccgagcaaacaccggcagccaactgagaatccaacgcgcagacgcccacattctccgcaccgcggccatccaggtggcgctgcatccgatccgtcaagatccgttagcatttgtgtaa

SEQ ID NO: 107 - protein, 357 aa, Corynebacterium glutamicum
MFMLAQRTLPIHITAPHLPVARVFHQIRATDADRTSLQRDLELSQAGITRHVSALIDAGLVEETRVDSGARSGRPRTKLGIDGRHLTAWGVHIGLRSTDFAVCDLAGRVIRYERVDHEVSHSTPSETLNFVAHRLQTLSAGLPEPRNVGVALSAHLSANGTVTSEDYGWSEVEIGIHLPFPATIGSGVAAMAGSEIINAPLTQSTQSTLYFYAREMVSHAWIFNGAVHRPNSGRTPTAFGNTNTLKDAFRRGLTPTTFSDLVQLSHTNPLARQILNERAHKLADAVTTAVDVVDPEAVVFAGEAFTLDPETLRIVVTQLRANTGSQLRIQRADAHILRTAAIQVALHPIRQDPLAFV

SEQ ID NO: 108 - DNA, 2180 bp, Artificial Sequence
  promoter P2
tttcgcggtgaatcaacccacccgaacggcgatccttcgaagtattttgccgattgatcaattagcgtcggcaacatcactgaatatgctgctcatgcagaccggcgcaatcgttggcccgctgatcgcaggtgcgttgattccgctgatcggtttcgggtggctgtatttccttgatgttgtctccatcatccccacactgtgggctgtatggtcactgccttcaatcaagccatccggcaaggtcatgaaggccggtttcgccagtgtggtggatggcctgaagtatttggctggccaacccgtgttgttgatggtgatggtgctggatcttatcgccatgattttcggcatgccacgtgcgctttaccccgagatcgcggaagtgaacttcggtggtggtgacgccggtgcaacgatgctggcgttcatgtactcatccatggctgttggcgcagttcttggcggcgtgctgtctggttgggtttcccggattagccgccagggtgttgcagtttattggtgcatcatcgcctggggcgcagccgttgctttgggtggcgtagcaattgttgtcagccccggcgctgtgaccgcgtgggcgtggatgttcatcatcatgatggtcattggtggcatggctgacatgtttagctcggctgttcgaaatgctattttgcagcagtctgcagcggaacatgtgcagggccgaatccaaggtgtgtggatcatcgtcgtggtgggtggacctcgtttagctgacgtccttcacggttgggccgctgagcccttgggtgcaggttggacggtattatggggcggagtagcggtggttgtactcactgcaatttgtatggtggcggtgcctaaattctggaaatacgagaaaccaaaaattaccggcatctaaatacttatccatgcccatttacagacaatgccttagctttgacctgcacaaatagttgcaaattgtcccacatacacataaagtagcttgcgtatttaaaattatgaacctaaggggtttagcaatgcccaatcaggcccacttctctgcgtcctttgcccgcccctctaccccggctgcaaagtgcatgcaccatatccgcctcggccagcaactcattagaaatgagctggtcgaggccacaggtctgtcccaaccgactgtcacccgcgcagtcaccgctttaatgcaggcaggtttggttcgtgaacgccctgatctcacactctcatcgggccctggtcgtcccaatattcctctagaactcgctccaagtccatggattcatgcaggcgtggcaatcggcaccaagtcttcctacgtcgctttgtttgataccaagggtcgcacccttcgtgatgccatactggaaatctcagcagctgatttagatccagacaccttcatcgaacacctcatcgctggtgtcaaccgcctcaccactggtcttgatctaccactggtaggtattggtgtggctacctcaggaaaagtcaccaacgcgggcgttgtcaccgcaagcaacttgggctgggatggcgttgatatcgccggccgtctgaactaccaattcagcgttccagcaaccgtggcatcagcaattcctgccatcgcagcttctgaactgcaggcttccccacttccccaccctgagcagccaactcccatcaccttgaccttctacgccgatgactctgtgggcgcggcctacagcaatgatttgggagtacatgtcattggaccactggctacaactcgtggatcaggtttggatactttgggcatggctgctgaagatgcgctgagcacccaaggtttcttaagcagggtttctgatcagggtatctttgccaacagccttggtgagctagtcaccattgctaaagacaatgaaaccgcacgggaattcctcaacgatcgcgcgaccctgctggctcacactgccgcagaagctgctgaaacagttaagccatccaccctggttctctcgggatcggcgttttccgaagatccacaaggtcggttggtgttcgcttcccaattgaagaaggaatacgacgcagacattgagctccgcttgatccccacccaccgggaaaatgtccgcgcagcagctcgcgcagtcgcacttgatcgactactcaacgagccacttaccctcgtaccctaa

SEQ ID NO: 109 - DNA, 2247 bp, Artificial Sequence
  promoter P4
ccctcatgagttcaggggttagaaaagcaatgggatttggatgcggttcggttttggccgtcatcatggttatctcatttgttggatgggcgcttagcttcatggatggaacggcacctattcgccaactccagcaaatccctgaagatgttccgccggcgcgtggtgtagaagttccgcaaattgatacaggggcagatggacgcacgtcagatcatttgcgtttttgggcggaaccaattgctcaagatgctggtgtgtccgctcaagcgattgcggcttatggaaacgcagagctcattgcgagtactgcgtggcctggctgcaatctggggtggaataccttggcaggtatcggccaggtggaaacccgtcacggtacctacaacggcaaaatgttcgggggcagttccctggatgaaaatggagttgcaacccctccaatcatcggcgttccacttgatggttcaccggggtttgcggaaattcccgacactgatggtggggaattagatggcgatactgaatatgatcgcgcggtaggtcccatgcagttcattccggaaacgtggcgacttatgggattggatgcaaacggtgatggggtagcggaccccaaccaaattgatgacgcagcattgagtgccgcaaacctgttgtgttccaacgatcgtgacttgtccactcctgaaggatggaccgcagctgttcattcttacaacatgtctaatcagtatttgatggacgttcgagatgctgccgcgtcctacgctttacgacagccggcgatctaaaacttaacaagcgcaacccccgaaaatgtgagattatgtccggtcggacacgtgcgggctggggatatgggtagtttaataaatttataccacacagtctattgcaatagaccaagctgttcagtagggtgcatgggagaagaatttcctaataaaaactcttaaggacctccaagtggctgaaatcatgcacgtattcgctcgcgaaattctcgactcccgcggtaacccaaccgtcgaggcagaggttttccttgatgacggttcccacggtgtcgcaggtgttccatccggcgcatccaccggcgtccacgaggctcatgagctgcgtgacggtggcgatcgctacctgggcaagggcgttttgaaggcagttgaaaacgtcaacgaagaaatcggcgacgagctcgctggcctagaggctgacgatcagcgcctcatcgacgaagcaatgatcaagcttgatggcaccgccaacaagtcccgcctgggtgcaaacgcaatccttggtgtttccatggctgttgcaaaggctgctgctgattccgcaggcctcccactgttccgctacatcggtggaccaaacgcacacgttcttccagttccaatgatgaacatcatcaacggtggcgctcacgctgactccggtgttgacgttcaggaattcatgatcgctccaatcggtgcagagaccttctctgaggctctccgcaacggcgcagaggtctaccacgcactgaagtccgtcatcaaggaaaagggcctgtccaccggacttggcgatgagggcggcttcgctccttccgtcggctccacccgtgaggctcttgaccttatcgttgaggcaatcgagaaggctggcttcaccccaggcaaggacatcgctcttgctctggacgttgcttcctctgagttcttcaaggacggcacctaccacttcgaaggtggccagcactccgcagctgagatggcaaacgtttacgctgagctcgttgacgcgtacccaatcgtctccatcgaggacccactgcaggaagatgactgggagggttacaccaacctcaccgcaaccatcggcgacaaggttcagatcgttggcgacgacttcttcgtcaccaaccctgagcgcctgaaggagggcatcgctaagaaggctgccaactccatcctggttaaggtgaaccagatcggtaccctcaccgagaccttcgacgctgtcgacatggctcaccgcgcaggctacacctccatgatgtcccaccgttccggtgagaccgaggacaccaccattgctgacctcgcagttgcactcaactgtggccagatcaagactggtgctccagcacgttccgaccgtgtcgcaaagtacaaccagcttctccgcatcgagcagttgcttggcgacgccggcgtctacgcaggtcgcagcgcattcccacgctttcagggctaa

SEQ ID NO: 110 - DNA, 2192 bp, Artificial Sequence
  promoter P8
tcaccgagtctttgatcaagggtggcgcttttgactcccttggacacgcacgaaaaggcctcatgctggtcttcgaagatgccgttgattccgtcatcgctaccaaaaaagctgctgacaagggacaatttgatctctttgcagctttcgactcggataacaacgacgatgtggcaagtttcttccagatcaccgttcctgatgacgaatgggaccgtaagcatgagctcgcactcgagcgagaaatgctgggtctgtatgtttctggacacccactcgatggctatgaagatgccattgctgcccaggttgatacagcactgaccaccattgttgccggtgaactcaagcacggcgcagaagtgaccgtgggtggcattatctctggtgtggatcgacggttctccaagaaggacggttccccttgggcgattgtcaccattgaagatcacaacggcgcgtccgttgaattgttggtcttcaacaaggtgtattccatcgttggatccatgattgtggaagacaacatcattttggccaaggcacacatctccattcgagatgatcgtatgagccttttctgtgatgatctccgcgttccagagcttgggccaggaaacgggcaaggacttccgcttcgtttgtccatgcgtactgatcagtgcaccatgtccaacattgccaagctcaagcaggtgctggtggacaacaagggtgaatctgatgtgtacctcaatttgatcgatggggataactccacggtcatgattttgggtgatcacttaagagtcaaccgatccgcaagtttgatgggcgacctcaaggcaacgatggggccaggcatcctcggttaatcacatcacactgggattaccccgtgtaggggtgaaaacccgaatgtggctaaaacttttggaaacttaagttacctttaatcggaaacttattgaattcgggtgaggcaactgcaactctggacttaaagcatgagccagaaccgcatcaggaccactcacgttggttccttgccccgtaccccagagctacttgatgcaaacatcaagcgctctaacggtgagattggggaggaggaattcttccagatcctgcagtcttctgtagatgacgtgatcaagcgccaggttgacctgggtatcgacatcctcaacgagggcgaatacggccacgtcacctccggtgcagttgacttcggtgcatggtggaactactccttcacccgcctgggcggactgaccatgaccgataccgaccgttgggcaagccaggaagcagtgcgttccacccctggcaacatcaagctgaccagcttctctgatcgtcgcgaccgcgcattgttcagcgaagcatacgaggatccagtatctggcatcttcaccggccgcgcttctgtgggcaacccagagttcaccggacctattacctacattggccaggaagaaactcagacggatgttgatctgctgaagaagggcatgaacgcagcgggagctaccgacggcttcgttgcagcactatccccaggatctgcagctcgattgaccaacaagttctacgacactgatgaagaagtcgtcgcagcatgtgccgatgcgctttcccaggaatacaagatcatcaccgatgcaggtctgaccgttcagctcgacgcaccggacttggcagaagcatgggatcagatcaacccagagccaagcgtgaaggattacttagactggatcggtacacgcatcgatgccatcaacagtgcagtgaagggccttccaaaggaacagacccgcctgcacatctgctggggctcttggcacggaccacacgtcactgacatcccattcggtgacatcattggtgagatcctgcgcgcagaggtcggtggcttctccttcgaaggcgcatctcctcgtcacgcacacgagtggcgtgtatgggaagaaaacaagcttcctgaaggctctgttatctaccctggtgttgtgtctcactccatcaacgctgtggagcacccacgcctggttgctgatcgtatcgttcagttcgccaagcttgttggccctgagaacgtcattgcgtccactgactgtggtctgggcggacgtctgcattcccagatcgcatgggcaaagctggagtccctagtagagggcgctcgcattgcatcaaaggaactgttctaa

SEQ ID NO: 111 - DNA, 97 bp, Artificial Sequence
  promoter P3
tgccgtttctcgcgttgtgtgtggtactacgtggggacctaagcgtgtaagatggaaacgtctgtatcggataagtagcgaggagtgttcgttaaaa

SEQ ID NO: 112 - DNA, 35 bp, Artificial Sequence
  primer
ccaagcttgcatgcctcaccgagtctttgatcaag

SEQ ID NO: 113 - DNA, 35 bp, Artificial Sequence
  primer
caaaagttttagccacattcgggttttcaccccta

SEQ ID NO: 114 - DNA, 35 bp, Artificial Sequence
  primer
ctctggacttaaagcatgagccagaaccgcatcag

SEQ ID NO: 115 - DNA, 35 bp, Artificial Sequence
  primer
cggtacccggggatcttagaacagttcctttgatg

SEQ ID NO: 116 - DNA, 87 bp, Artificial Sequence
  DNA fragment of P8 promoter
gtggctaaaacttttggaaacttaagttacctttaatcggaaacttattgaattcgggtgaggcaactgcaactctggacttaaagc

SEQ ID NO: 117 - DNA, 35 bp, Artificial Sequence
  primer
gtgaaaacccgaatgtggctaaaacttttggaaac

SEQ ID NO: 118 - DNA, 35 bp, Artificial Sequence
  primer
gcggttctggctcatgctttaagtccagagttgca

SEQ ID NO: 119 - DNA, 1206 bp, Corynebacterium glutamicum
atgagccagaaccgcatcaggaccactcacgttggttccttgccccgtaccccagagctacttgatgcaaacatcaagcgttctaacggtgagattggggaggaggaattcttccagattctgcagtcttctgtagatgacgtgatcaagcgccaggttgacctgggtatcgacatccttaacgagggcgaatacggccacgtcacctccggtgcagttgacttcggtgcatggtggaactactccttcacccgcctgggcggactgaccatgaccgataccgaccgttgggcaagccaggaagcagtgcgttccacccctggcaacatcaagctgaccagcttctctgatcgtcgcgaccgcgcattgttcagcgaagcatacgaggatccagtatctggcatcttcaccggtcgcgcttctgtgggcaacccagagttcaccggacctattacctacattggccaggaagaaactcagacggatgttgatctgctgaagaagggcatgaacgcagcgggagctaccgacggcttcgttgcagcactatccccaggatctgcagctcgattgaccaacaagttctacgacactgatgaagaagtcgtcgcagcatgtgctgatgcgctttcccaggaatacaagatcatcaccgatgcaggtctgaccgttcagctcgacgcaccggacttggcagaagcatgggatcagatcaacccagagccaagcgtgaaggattacttggactggatcggtacacgcatcgatgccatcaacagtgcagtgaagggccttccaaaggaacagacccgcctgcacatctgctggggctcttggcacggaccacacgtcactgacatcccattcggtgacatcattggtgagatcctgcgcgcagaggtcggtggcttctccttcgaaggcgcatctcctcgtcacgcacacgagtggcgtgtatgggaagaaaacaagcttcctgaaggctctgttatctaccctggtgttgtgtctcactccatcaacgctgtggagcacccacgcctggttgctgatcgtatcgttcagttcgccaagcttgttggccctgagaacgtcattgcgtccactgactgtggtctgggcggacgtctgcattcccagatcgcatgggcaaagctggagtccctagtagagggcgctcgcattgcatcaaaggaactgttctaa

SEQ ID NO: 120 - protein, 401 aa, Corynebacterium glutamicum
MSQNRIRTTHVGSLPRTPELLDANIKRSNGEIGEEEFFQILQSSVDDVIKRQVDLGIDILNEGEYGHVTSGAVDFGAWWNYSFTRLGGLTMTDTDRWASQEAVRSTPGNIKLTSFSDRRDRALFSEAYEDPVSGIFTGRASVGNPEFTGPITYIGQEETQTDVDLLKKGMNAAGATDGFVAALSPGSAARLTNKFYDTDEEVVAACADALSQEYKIITDAGLTVQLDAPDLAEAWDQINPEPSVKDYLDWIGTRIDAINSAVKGLPKEQTRLHICWGSWHGPHVTDIPFGDIIGEILRAEVGGFSFEGASPRHAHEWRVWEENKLPEGSVIYPGVVSHSINAVEHPRLVADRIVQFAKLVGPENVIASTDCGLGGRLHSQIAWAKLESLVEGARIASKELF

SEQ ID NO: 121 - DNA, 35 bp, Artificial Sequence
  primer
ccaagcttgcatgccccctcatgagttcaggggtt

SEQ ID NO: 122 - DNA, 35 bp, Artificial Sequence
  primer
tggtataaatttattaaactacccatatccccagc

SEQ ID NO: 123 - DNA, 35 bp, Artificial Sequence
  primer
cttaaggacctccaagtggctgaaatcatgcacgt

SEQ ID NO: 124 - DNA, 35 bp, Artificial Sequence
  primer
cggtacccggggatcttagccctgaaagcgtggga

SEQ ID NO: 125 - DNA, 98 bp, Artificial Sequence
  DNA fragment of P4 promoter
aataaatttataccacacagtctattgcaatagaccaagctgttcagtagggtgcatgggagaagaatttcctaataaaaactcttaaggacctccaa

SEQ ID NO: 126 - DNA, 35 bp, Artificial Sequence
  primer
ggatatgggtagtttaataaatttataccacacag

SEQ ID NO: 127 - DNA, 35 bp, Artificial Sequence
  primer
catgatttcagccacttggaggtccttaagagttt

SEQ ID NO: 128 - DNA, 1278 bp, Corynebacterium glutamicum
gtggctgaaatcatgcacgtattcgctcgcgaaattctcgactcccgcggtaacccaaccgtcgaggcagaggttttccttgatgacggttcccacggtgtcgcaggtgttccatccggcgcatccaccggcgtccacgaggctcatgagctgcgtgacggtggcgatcgctacctgggcaagggcgttttgaaggcagttgaaaacgtcaacgaagaaatcggcgacgagctcgctggcctagaggctgacgatcagcgcctcatcgacgaagcaatgatcaagcttgatggcaccgccaacaagtcccgcctgggtgcaaacgcaatccttggtgtttccatggctgttgcaaaggctgctgctgattccgcaggcctcccactgttccgctacatcggtggaccaaacgcacacgttcttccagttccaatgatgaacatcatcaacggtggcgctcacgctgactccggtgttgacgttcaggaattcatgatcgctccaatcggtgcagagaccttctctgaggctctccgcaacggcgcagaggtctaccacgcactgaagtccgtcatcaaggaaaagggcctgtccaccggacttggcgatgagggcggcttcgctccttccgtcggctccacccgtgaggctcttgaccttatcgttgaggcaatcgagaaggctggcttcaccccaggcaaggacatcgctcttgctctggacgttgcttcctctgagttcttcaaggacggcacctaccacttcgaaggtggccagcactccgcagctgagatggcaaacgtttacgctgagctcgttgacgcgtacccaatcgtctccatcgaggacccactgcaggaagatgactgggagggttacaccaacctcaccgcaaccatcggcgacaaggttcagatcgttggcgacgacttcttcgtcaccaaccctgagcgcctgaaggagggcatcgctaagaaggctgccaactccatcctggttaaggtgaaccagatcggtaccctcaccgagaccttcgacgctgtcgacatggctcaccgcgcaggctacacctccatgatgtcccaccgttccggtgagaccgaggacaccaccattgctgacctcgcagttgcactcaactgtggccagatcaagactggtgctccagcacgttccgaccgtgtcgcaaagtacaaccagcttctccgcatcgagcagttgcttggcgacgccggcgtctacgcaggtcgcagcgcattcccacgctttcagggctaa

SEQ ID NO: 129 - protein, 425 aa, Corynebacterium glutamicum
MAEIMHVFAREILDSRGNPTVEAEVFLDDGSHGVAGVPSGASTGVHEAHELRDGGDRYLGKGVLKAVENVNEEIGDELAGLEADDQRLIDEAMIKLDGTANKSRLGANAILGVSMAVAKAAADSAGLPLFRYIGGPNAHVLPVPMMNIINGGAHADSGVDVQEFMIAPIGAETFSEALRNGAEVYHALKSVIKEKGLSTGLGDEGGFAPSVGSTREALDLIVEAIEKAGFTPGKDIALALDVASSEFFKDGTYHFEGGQHSAAEMANVYAELVDAYPIVSIEDPLQEDDWEGYTNLTATIGDKVQIVGDDFFVTNPERLKEGIAKKAANSILVKVNQIGTLTETFDAVDMAHRAGYTSMMSHRSGETEDTTIADLAVALNCGQIKTGAPARSDRVAKYNQLLRIEQLLGDAGVYAGRSAFPRFQG

SEQ ID NO: 130 - DNA, 666 bp, Niastella koreensis
atgaataatcaaatttttgaatccgttgaccattatatcagcgatttactgggttacgaagacgatgcattgcttgccgccaccaattcattagccgaagcaggcatgcctgccatcagcgtatcacccaaccagggcaagtttctgcaattactggcccaattgtgccaggcaaaaaatatcctggagctgggcacactggcaggctacagcaccatttggatggcccgggccttacccaaaaacggccggctcatcacccttgaatatgaccccaaacatgcggccgttgcacaaaaaaatatcgaccgggccggccttacttcacaagtacagatcagaaccggtaaagcaattgacatattaccgcaattagtggaagaaggcgccggaccttttgatatgatctttatcgatgccgataaaccaccttacaccgaatattttcaatgggcgcttcggttatcacgtcccggtacactcatcgtggccgataatgtgatccgtgatggcaaagtgctggatgaaaacagtacggagcctgctgtacagggcgcaagacgtttcaatgccatgctgggcgccaataccgccgttgacgccaccattcttcaaatggtaggtgtaaaagaatacgatggaatggctttggccatagtaaaataa

SEQ ID NO: 131 - protein, 221 aa, Niastella koreensis
MNNQIFESVDHYISDLLGYEDDALLAATNSLAEAGMPAISVSPNQGKFLQLLAQLCQAKNILELGTLAGYSTIWMARALPKNGRLITLEYDPKHAAVAQKNIDRAGLTSQVQIRTGKAIDILPQLVEEGAGPFDMIFIDADKPPYTEYFQWALRLSRPGTLIVADNVIRDGKVLDENSTEPAVQGARRFNAMLGANTAVDATILQMVGVKEYDGMALAIVK

SEQ ID NO: 132 - DNA, 50 bp, Artificial Sequence
  primer
catgattacgccaagcttgcatgccaaattcctgtgattagctgatttag

SEQ ID NO: 133 - DNA, 50 bp, Artificial Sequence
  primer
cggattcgaagatctggttgttcatagaggcgaaggctccttgaataggt

SEQ ID NO: 134 - DNA, 778 bp, Niastella koreensis
atgaacaaccagatcttcgaatccgtcgatcactatatttctgatcttctgggctacgaggatgatgcgcttttggccgccactaattccctggccgaggcaggtatgccggctattagcgtttccccgaaccagggcaaatttttgcaactgctggcccaactttgccaagccaaaaacattttggagcttggtacgttggccggctattcgaccatctggatggctcgcgctctccccaagaacggccgccttatcaccctggaatacgatccgaagcatgccgcggtagctcagaagaacattgatcgcgctggcttgaccagccaagtgcaaatccgcacgggtaaagcaatcgacatcctgccgcagctggtggaggagggtgccggtccatttgatatgatcttcattgatgccgataagcccccatacaccgaatactttcaatgggctctgcgactgtcccgccccggcactctcatcgtcgcggataatgtcatccgcgatggaaaggtgctggacgaaaactccaccgagcctgccgtccaaggtgcccgccgttttaatgccatgctcggtgctaatacggcagttgacgcaaccatcctccaaatggtgggcgtgaaagagtacgacggcatggcgctggccatcgttaagtaaaagcttgcggccgcactcgagcaccaccaccaccaccactgagatccggctgctaacaaagcccgaaaggaagctgagttggctgctgccaccgctgagcaataactagcat

SEQ ID NO: 135 - DNA, 666 bp, Niastella koreensis
atgaacaaccagatcttcgaatccgtcgatcactatatttctgatcttctgggctacgaggatgatgcgcttttggccgccactaattccctggccgaggcaggtatgccggctattagcgtttccccgaaccagggcaaatttttgcaactgctggcccaactttgccaagccaaaaacattttggagcttggtacgttggccggctattcgaccatctggatggctcgcgctctccccaagaacggccgccttatcaccctggaatacgatccgaagcatgccgcggtagctcagaagaacattgatcgcgctggcttgaccagccaagtgcaaatccgcacgggtaaagcaatcgacatcctgccgcagctggtggaggagggtgccggtccatttgatatgatcttcattgatgccgataagcccccatacaccgaatactttcaatgggctctgcgactgtcccgccccggcactctcatcgtcgcggataatgtcatccgcgatggaaaggtgctggacgaaaactccaccgagcctgccgtccaaggtgcccgccgttttaatgccatgctcggtgctaatacggcagttgacgcaaccatcctccaaatggtgggcgtgaaagagtacgacggcatggcgctggccatcgttaagtaa

SEQ ID NO: 136 - DNA, 33 bp, Artificial Sequence
  primer
ctggccgaggcaggtaagccggctattagcgtt

SEQ ID NO: 137 - DNA, 33 bp, Artificial Sequence
  primer
aacgctaatagccggcttacctgcctcggccag

SEQ ID NO: 138 - DNA, 35 bp, Artificial Sequence
  primer
ccaagcttgcatgccggtaggtggcgtatcagact

SEQ ID NO: 139 - DNA, 35 bp, Artificial Sequence
  primer
acgcgagaaacggcactagttgagggcctctaaat

SEQ ID NO: 140 - DNA, 35 bp, Artificial Sequence
  primer
gagtgttcgttaaaaatggcacaggttatggactt

SEQ ID NO: 141 - DNA, 35 bp, Artificial Sequence
  primer
cggtacccggggatcttagtagcggtagtgctccg

SEQ ID NO: 142 - DNA, 35 bp, Artificial Sequence
  primer
gaggccctcaactagtgccgtttctcgcgttgtgt

SEQ ID NO: 143 - DNA, 35 bp, Artificial Sequence
  primer
cataacctgtgccatttttaacgaacactcctcgc

SEQ ID NO: 144 - DNA, 1437 bp, Corynebacterium glutamicum
atggcacaggttatggacttcaaggttgccgatctttcactagcagaggcaggacgtcaccagattcgtcttgcagagtatgagatgccaggtctcatgcagttgcgcaaggaattcgcagacgagcagcctttgaagggcgcccgaattgctggttccatccacatgacggtccagaccgccgtgcttattgagaccctcactgctttgggcgctgaggttcgttgggcttcctgcaacattttctccacccaggatgaggctgcagcggctatcgttgtcggctccggcaccgtcgaagagccagctggtgttccagtattcgcgtggaagggtgagtcactggaggagtactggtggtgcatcaaccagatcttcagctggggcgatgagctgccaaacatgatcctcgacgacggcggtgacgccaccatggctgttattcgcggtcgcgaatacgagcaggctggtctggttccaccagcagaggccaacgattccgatgagtacatcgcattcttgggcatgctgcgtgaggttcttgctgcagagcctggcaagtggggcaagatcgctgaggccgttaagggtgtcaccgaggaaaccaccaccggtgtgcaccgcctgtaccacttcgctgaagaaggcgtactgcctttcccagcgatgaacgtcaacgacgctgtcaccaagtccaagtttgataacaagtacggcacccgccactccctgatcgacggcatcaaccgcgccaccgacatgctcatgggcggcaagaacgtgcttgtctgcggttacggtgatgtcggcaagggctgcgctgaggctttcgacggccagggcgctcgcgtcaaggtcaccgaagctgacccaatcaacgctcttcaggctctgatggatggctactctgtggtcaccgttgatgaggccatcgaggacgccgacatcgtgatcaccgcgaccggtaacaaggacatcatttccttcgagcagatgctcaagatgaaggatcacgctctgctgggcaacatcggtcactttgataatgagatcgatatgcattccctgttgcaccgcgacgacgtcacccgcaccacgatcaagccacaggtcgacgagttcaccttctccaccggtcgctccatcatcgtgctgtctgaaggccgtctgctaaaccttggcaacgccaccggacacccatcatttgtcatgtccaactctttcgccgatcagaccattgcgcagatcgaactgttccaaaacgaaggacagtacgagaacgaggtctaccgtctgcctaaggttctcgacgaaaaggtggcacgcatccacgttgaggctctcggcggtcagctcaccgaactgaccaaggagcaggctgagtacatcggcgttgacgttgcaggtccattcaagccggagcactaccgctactaa

SEQ ID NO: 145 - protein, 478 aa, Corynebacterium glutamicum
MAQVMDFKVADLSLAEAGRHQIRLAEYEMPGLMQLRKEFADEQPLKGARIAGSIHMTVQTAVLIETLTALGAEVRWASCNIFSTQDEAAAAIVVGSGTVEEPAGVPVFAWKGESLEEYWWCINQIFSWGDELPNMILDDGGDATMAVIRGREYEQAGLVPPAEANDSDEYIAFLGMLREVLAAEPGKWGKIAEAVKGVTEETTTGVHRLYHFAEEGVLPFPAMNVNDAVTKSKFDNKYGTRHSLIDGINRATDMLMGGKNVLVCGYGDVGKGCAEAFDGQGARVKVTEADPINALQALMDGYSVVTVDEAIEDADIVITATGNKDIISFEQMLKMKDHALLGNIGHFDNEIDMHSLLHRDDVTRTTIKPQVDEFTFSTGRSIIVLSEGRLLNLGNATGHPSFVMSNSFADQTIAQIELFQNEGQYENEVYRLPKVLDEKVARIHVEALGGQLTELTKEQAEYIGVDVAGPFKPEHYRY

SEQ ID NO: 146 - DNA, 20 bp, Artificial Sequence
  primer
gtccaactctttcgccgatc

SEQ ID NO: 147 - DNA, 20 bp, Artificial Sequence
  primer
gagaaccttaggcagacggt

SEQ ID NO: 148 - DNA, 20 bp, Artificial Sequence
  primer
caatcgagaaggctggcttc

SEQ ID NO: 149 - DNA, 20 bp, Artificial Sequence
  primer
gtgccgtccttgaagaactc

SEQ ID NO: 150 - DNA, 20 bp, Artificial Sequence
  primer
aggtggggatgacgtcaaat

SEQ ID NO: 151 - DNA, 20 bp, Artificial Sequence
  primer
gaactgaggccggctttaag